European Patent Application EP 4 616 914 A2, published September 17, 2025. Title: POLYPEPTIDES BINDING TO HUMAN COMPLEMENT C5. Applicant: IPC Research, LLC. Application EP. The sequence listing filed with the application follows.

SEQUENCE LISTING (765 sequences)

SEQ ID NO: 1 - protein, 29 aa, synthetic construct
  REGION 1..29: note = Modified bacterial sequence
EVLEAWDEIDRLPNLTIEQWLAFINKLDD

SEQ ID NO: 2 - protein, 29 aa, synthetic construct
  REGION 1..29: note = Modified bacterial sequence
EVLEAWNEIDRLPNLTIEQWLAFINKLDD

SEQ ID NO: 3 - protein, 29 aa, synthetic construct
  REGION 1..29: note = Modified bacterial sequence
EVIEAWNEIDRLPNLTIEQWLAFINKLDD

SEQ ID NO: 4 - protein, 29 aa, synthetic construct
  REGION 1..29: note = Modified bacterial sequence
EVLEAWDEIDRLPNLTLDQWLAFINKLDD

SEQ ID NO: 5 - protein, 29 aa, synthetic construct
  REGION 1..29: note = Modified bacterial sequence
EVLDAWDEIDALPNLTLEQWLAFINKLDD

SEQ ID NO: 6 - protein, 29 aa, synthetic construct
  REGION 1..29: note = Modified bacterial sequence
EVIDAWDEIDRLPNLTLDQWLAFINKLDD

SEQ ID NO: 7 - protein, 29 aa, synthetic construct
  REGION 1..29: note = Modified bacterial sequence
ETLEAWDEIDRLPNLTIEQWLAFINKLDD

SEQ ID NO: 8 - protein, 29 aa, synthetic construct
  REGION 1..29: note = Modified bacterial sequence
EVIDAWNEIDALPNLTLDQWLAFINKLDD

SEQ ID NO: 9 - protein, 29 aa, synthetic construct
  REGION 1..29: note = Modified bacterial sequence
EVLDAWDEIDKLPNLTIDQWLAFINKLDD

SEQ ID NO: 10 - protein, 29 aa, synthetic construct
  REGION 1..29: note = Modified bacterial sequence
EVLEAWDEIDHLPNLTLDQWLAFINKLDD

SEQ ID NO: 11 - protein, 29 aa, synthetic construct
  REGION 1..29: note = Modified bacterial sequence
EVLEAWDEIDALPNLTIEQWLAFINKLDD

SEQ ID NO: 12 - protein, 29 aa, synthetic construct
  REGION 1..29: note = Modified bacterial sequence
EVLDAWDEIDKLPNLTLEQWLAFINKLDD

SEQ ID NO: 13 - protein, 29 aa, synthetic construct
  REGION 1..29: note = Modified bacterial sequence
ETITAWDEIDKLPNLTIEQWLAFIGKLED

SEQ ID NO: 14 - protein, 29 aa, synthetic construct
  REGION 1..29: note = Modified bacterial sequence
ESMKAWDEIDRLPNLNINQWVAFIDSLYD

SEQ ID NO: 15 - protein, 29 aa, synthetic construct
  REGION 1..29: note = Modified bacterial sequence
ESIEAWTEIDHLPNLTIEQWLAFINKLTD

SEQ ID NO: 16 - protein, 29 aa, synthetic construct
  REGION 1..29: note = Modified bacterial sequence
EVLDAWHEIDTLPNLTVRQWLAFISKLED

SEQ ID NO: 17 - protein, 29 aa, synthetic construct
  REGION 1..29: note = Modified bacterial sequence
EHIQANEEIDRLPNLTIKQWLAFINKLHD

SEQ ID NO: 18 - protein, 29 aa, synthetic construct
  REGION 1..29: note = Modified bacterial sequence
EVLHAWAEIDALPNLTIEQWLAFINKLDD

SEQ ID NO: 19 - protein, 29 aa, synthetic construct
  REGION 1..29: note = Modified bacterial sequence
EVLAAWDEIDSLPNLTLQQWLAFINKLDD

SEQ ID NO: 20 - protein, 29 aa, synthetic construct
  REGION 1..29: note = Modified bacterial sequence
EVIDAWNEIDALPNLTLEQWLAFINKLDD

SEQ ID NO: 21 - protein, 29 aa, synthetic construct
  REGION 1..29: note = Modified bacterial sequence
EVLDAWNEIDALPNLTIDQWLAFINKLSD

SEQ ID NO: 22 - protein, 29 aa, synthetic construct
  REGION 1..29: note = Modified bacterial sequence
EVIEAWDEIDGLPNLTIEQWLAFINKLDD

SEQ ID NO: 23 - protein, 29 aa, synthetic construct
  REGION 1..29: note = Modified bacterial sequence
EVLEAWDEIDHLPNLTLQQWLAFINKLDD

SEQ ID NO: 24 - protein, 29 aa, synthetic construct
  REGION 1..29: note = Modified bacterial sequence
EVIEAWNEIDALPNLTIEQWLAFINKLDD

SEQ ID NO: 25 - protein, 29 aa, synthetic construct
  REGION 1..29: note = Modified bacterial sequence
EVIAAWNEIDRLPNLTLTQWLAFINKLDD

SEQ ID NO: 26 - protein, 29 aa, synthetic construct
  REGION 1..29: note = Modified bacterial sequence
EVIEAWDEIDALPNLTLQQWLAFINKLDD

SEQ ID NO: 27 - protein, 29 aa, synthetic construct
  REGION 1..29: note = Modified bacterial sequence
EVIAAWDEIDKLPNLTIEQWLAFINKLDD

SEQ ID NO: 28 - protein, 29 aa, synthetic construct
  REGION 1..29: note = Modified bacterial sequence
EVIAAWDEIDKLPNLTLQQWLAFINKLDD

SEQ ID NO: 29 - protein, 29 aa, synthetic construct
  REGION 1..29: note = Modified bacterial sequence
ETIAAWDEIDKLPNLTIEQWLAFINKLDD

SEQ ID NO: 30 - protein, 29 aa, synthetic construct
  REGION 1..29: note = Modified bacterial sequence
ETIEAWNEIDRLPNLTIEQWLAFINKLDD

SEQ ID NO: 31 - protein, 29 aa, synthetic construct
  REGION 1..29: note = Modified bacterial sequence
EVLEAWREIDALPNLTIQQWLAFINKLDD

SEQ ID NO: 32 - protein, 29 aa, synthetic construct
  REGION 1..29: note = Modified bacterial sequence
EVIEAWDEIDQLPNLTIEQWLAFINKLDD

SEQ ID NO: 33 - protein, 29 aa, synthetic construct
  REGION 1..29: note = Modified bacterial sequence
EVLRAWDEIDHLPNLTLEQWLAFINKLDD

SEQ ID NO: 34 - protein, 29 aa, synthetic construct
  REGION 1..29: note = Modified bacterial sequence
EVLEAWDEIDRLPNLTLNQWLAFINKLDD

SEQ ID NO: 35 - protein, 29 aa, synthetic construct
  REGION 1..29: note = Modified bacterial sequence
EVLDAWNEIDHLPNLTIEQWLAFINKLDD

SEQ ID NO: 36 - protein, 29 aa, synthetic construct
  REGION 1..29: note = Modified bacterial sequence
EVIDAWNEIDKLPNLTIEQWLAFINKLDD

SEQ ID NO: 37 - protein, 29 aa, synthetic construct
  REGION 1..29: note = Modified bacterial sequence
ETLEAWDEIDQLPNLTLQQWLAFINKLDD

SEQ ID NO: 38 - protein, 29 aa, synthetic construct
  REGION 1..29: note = Modified bacterial sequence
EVIEAWNEIDALPNLTLDQWLAFINKLDD

SEQ ID NO: 39 - protein, 29 aa, synthetic construct
  REGION 1..29: note = Modified bacterial sequence
EVIDAWNEIDRLPNLTLQQWLAFINKLDD

SEQ ID NO: 40 - protein, 29 aa, synthetic construct
  REGION 1..29: note = Modified bacterial sequence
EVIDAWNEIDQLPNLTLEQWLAFINKLDD

SEQ ID NO: 41 - protein, 29 aa, synthetic construct
  REGION 1..29: note = Modified bacterial sequence
ETIAAWDEIDHLPNLTLEQWLAFINKLDD

SEQ ID NO: 42 - protein, 29 aa, synthetic construct
  REGION 1..29: note = Modified bacterial sequence
EVLQAWDEIDHLPNLTIQQWLAFINKLSD

SEQ ID NO: 43 - protein, 29 aa, synthetic construct
  REGION 1..29: note = Modified bacterial sequence
ETLHAWAEIDRLPNLTIEQWLAFINKLDD

SEQ ID NO: 44 - protein, 29 aa, synthetic construct
  REGION 1..29: note = Modified bacterial sequence
EVLEAWNEIDHLPNLTLAQWLAFINKLDD

SEQ ID NO: 45 - protein, 29 aa, synthetic construct
  REGION 1..29: note = Modified bacterial sequence
EVIEAWDEIDKLPNLTIAQWLAFINKLDD

SEQ ID NO: 46 - protein, 29 aa, synthetic construct
  REGION 1..29: note = Modified bacterial sequence
EVLDAWDEIDHLPNLTLQQWLAFINKLDD

SEQ ID NO: 47 - protein, 29 aa, synthetic construct
  REGION 1..29: note = Modified bacterial sequence
ETIEAWNEIDKLPNLTLTQWLAFINKLDD

SEQ ID NO: 48 - protein, 29 aa, synthetic construct
  REGION 1..29: note = Modified bacterial sequence
EVLEAWNEIDLLPNLTIEQWLAFINKLDD

SEQ ID NO: 49 - protein, 29 aa, synthetic construct
  REGION 1..29: note = Modified bacterial sequence
EVIEAWDEIDHLPNLTIDQWLAFINKLDD

SEQ ID NO: 50 - protein, 29 aa, synthetic construct
  REGION 1..29: note = Modified bacterial sequence
EVISAWNEIDALPNLTLQQWLAFINKLDD

SEQ ID NO: 51 - protein, 29 aa, synthetic construct
  REGION 1..29: note = Modified bacterial sequence
EVIAAWNEIDKLPNLTLEQWLAFINKLDD

SEQ ID NO: 52 - protein, 29 aa, synthetic construct
  REGION 1..29: note = Modified bacterial sequence
ETIEAWNEIDSLPNLTLDQWLAFINKLDD

SEQ ID NO: 53 - protein, 29 aa, synthetic construct
  REGION 1..29: note = Modified bacterial sequence
EVLDAWNEIDQLPNLTLQQWLAFINKLDD

SEQ ID NO: 54 - protein, 29 aa, synthetic construct
  REGION 1..29: note = Modified bacterial sequence
EVLAAWNEIDHLPNLTIEQWLAFINKLDD

SEQ ID NO: 55 - protein, 29 aa, synthetic construct
  REGION 1..29: note = Modified bacterial sequence
EVLEAWDEIDHLPNLTITQWLAFINKLDD

SEQ ID NO: 56 - protein, 29 aa, synthetic construct
  REGION 1..29: note = Modified bacterial sequence
ETIDAWNEIDHLPNLTIEQWLAFINKLDD

SEQ ID NO: 57 - protein, 29 aa, synthetic construct
  REGION 1..29: note = Modified bacterial sequence
EVIEAWNEIDHLPNLTIQQWLAFINKLDD

SEQ ID NO: 58 - protein, 29 aa, synthetic construct
  REGION 1..29: note = Modified bacterial sequence
EVIQAWNEIDALPNLTISQWLAFINKLDD

SEQ ID NO: 59 - protein, 29 aa, synthetic construct
  REGION 1..29: note = Modified bacterial sequence
EVIAAWDEIDSLPNLTIEQWLAFINKLDD

SEQ ID NO: 60 - protein, 29 aa, synthetic construct
  REGION 1..29: note = Modified bacterial sequence
EHIEAWNEIDALPNLTIEQWLAFINKLQD

SEQ ID NO: 61 - protein, 29 aa, synthetic construct
  REGION 1..29: note = Modified bacterial sequence
EVLEAWNEIDKLPNLTLDQWLAFINKLDD

SEQ ID NO: 62 - protein, 29 aa, synthetic construct
  REGION 1..29: note = Modified bacterial sequence
EVIDAWNEIDHLPNLTIEQWLAFINKLAD

SEQ ID NO: 63 - protein, 29 aa, synthetic construct
  REGION 1..29: note = Modified bacterial sequence
ETIDAWDEIDKLPNLTIEQWLAFINKLDD

SEQ ID NO: 64 - protein, 29 aa, synthetic construct
  REGION 1..29: note = Modified bacterial sequence
EVIAAWDEIDLLPNLTLQQWLAFINKLAD

SEQ ID NO: 65 - protein, 29 aa, synthetic construct
  REGION 1..29: note = Modified bacterial sequence
EVIHAWDEIDKLPNLTIEQWLAFINKLDD

SEQ ID NO: 66 - protein, 29 aa, synthetic construct
  REGION 1..29: note = Modified bacterial sequence
EVIAAWNEIDHLPNLTLEQWLAFINKLDD

SEQ ID NO: 67 - protein, 29 aa, synthetic construct
  REGION 1..29: note = Modified bacterial sequence
ETLDAWNEIDKLPNLTLSQWLAFINKLDD

SEQ ID NO: 68 - protein, 29 aa, synthetic construct
  REGION 1..29: note = Modified bacterial sequence
EVLEAWNEIDALPNLTLEQWLAFINKLDD

SEQ ID NO: 69 - protein, 29 aa, synthetic construct
  REGION 1..29: note = Modified bacterial sequence
EVIQAWDEIDHLPNLTISQWLAFINKLDD

SEQ ID NO: 70 - protein, 29 aa, synthetic construct
  REGION 1..29: note = Modified bacterial sequence
EVLQAWDEIDSLPNLTIEQWLAFINKLDD

SEQ ID NO: 71 - protein, 29 aa, synthetic construct
  REGION 1..29: note = Modified bacterial sequence
ETLEAWDEIDHLPNLTIAQWLAFINKLDD

SEQ ID NO: 72 - protein, 29 aa, synthetic construct
  REGION 1..29: note = Modified bacterial sequence
ETIDAWNEIDRLPNLTISQWLAFINKLDD

SEQ ID NO: 73 - protein, 29 aa, synthetic construct
  REGION 1..29: note = Modified bacterial sequence
EVLDAWHEIDHLPNLTIQQWLAFINKLDD

SEQ ID NO: 74 - protein, 29 aa, synthetic construct
  REGION 1..29: note = Modified bacterial sequence
EQIRAWDEIDKLPNLTIEQWLAFINKLAD

SEQ ID NO: 75 - protein, 29 aa, synthetic construct
  REGION 1..29: note = Modified bacterial sequence
ETLYAWNEIDKLPNLTIEQWLAFIEKLQD

SEQ ID NO: 76 - protein, 29 aa, synthetic construct
  REGION 1..29: note = Modified bacterial sequence
EVIEAWNEIDALPNLTIDQWLAFINKLDD

SEQ ID NO: 77 - protein, 29 aa, synthetic construct
  REGION 1..29: note = Modified bacterial sequence
EVLEAWNEIDHLPNLTIQQWLAFINKLDD

SEQ ID NO: 78 - protein, 29 aa, synthetic construct
  REGION 1..29: note = Modified bacterial sequence
ETIEAWDEIDALPNLTIEQWLAFINKLDD

SEQ ID NO: 79 - protein, 29 aa, synthetic construct
  REGION 1..29: note = Modified bacterial sequence
EVIEAWNEIDHLPNLTLQQWLAFINKLDD

SEQ ID NO: 80 - protein, 29 aa, synthetic construct
  REGION 1..29: note = Modified bacterial sequence
EVIEAWNEIDKLPNLTIQQWLAFINKLDD

SEQ ID NO: 81 - protein, 29 aa, synthetic construct
  REGION 1..29: note = Modified bacterial sequence
ETLDAWAEIDHLPNLTLDQWLAFINKLDD

SEQ ID NO: 82 - protein, 29 aa, synthetic construct
  REGION 1..29: note = Modified bacterial sequence
EHIDAWNEIDALPNLTLSQWLAFINKLDD

SEQ ID NO: 83 - protein, 29 aa, synthetic construct
  REGION 1..29: note = Modified bacterial sequence
EVLDAWNEIDKLPNLTIAQWLAFINKLDD

SEQ ID NO: 84 - protein, 29 aa, synthetic construct
  REGION 1..29: note = Modified bacterial sequence
EVIEAWTEIDYLPNLTLQQWLAFINKLDD

SEQ ID NO: 85 - protein, 29 aa, synthetic construct
  REGION 1..29: note = Modified bacterial sequence
ETIEAWNEIDHLPNLTIAQWLAFINKLDD

SEQ ID NO: 86 - protein, 29 aa, synthetic construct
  REGION 1..29: note = Modified bacterial sequence
EVIQAWNEIDKLPNLTLEQWLAFINKLDD

SEQ ID NO: 87 - protein, 29 aa, synthetic construct
  REGION 1..29: note = Modified bacterial sequence
EVIEAWDEIDHLPNLTIEQWLAFINKLDD

SEQ ID NO: 88 - protein, 29 aa, synthetic construct
  REGION 1..29: note = Modified bacterial sequence
ETIDAWNEIDLLPNLTIEQWLAFINKLDD

SEQ ID NO: 89 - protein, 29 aa, synthetic construct
  REGION 1..29: note = Modified bacterial sequence
EHIDAWNEIDKLPNLTLDQWLAFINKLDD

SEQ ID NO: 90 - protein, 29 aa, synthetic construct
  REGION 1..29: note = Modified bacterial sequence
EVVAAWNEIDALPNLTIEQWLAFINKLND

SEQ ID NO: 91 - protein, 29 aa, synthetic construct
  REGION 1..29: note = Modified bacterial sequence
EVIEAWNEIDALPNLTLAQWLAFINKLDD

SEQ ID NO: 92 - protein, 29 aa, synthetic construct
  REGION 1..29: note = Modified bacterial sequence
EVLQAWDEIDRLPNLTLDQWLAFINKLDD

SEQ ID NO: 93 - protein, 29 aa, synthetic construct
  REGION 1..29: note = Modified bacterial sequence
EVIDAWDEIDHLPNLTIEQWLAFINKLSD

SEQ ID NO: 94 - protein, 29 aa, synthetic construct
  REGION 1..29: note = Modified bacterial sequence
EVVEAWNEIDQLPNLTIEQWLAFINKLDD

SEQ ID NO: 95 - protein, 29 aa, synthetic construct
  REGION 1..29: note = Modified bacterial sequence
EVIQAWNEIDALPNLTIEQWLAFINKLDD

SEQ ID NO: 96 - protein, 29 aa, synthetic construct
  REGION 1..29: note = Modified bacterial sequence
EVIQAWDEIDKLPNLTIDQWLAFINKLAD

SEQ ID NO: 97 - protein, 29 aa, synthetic construct
  REGION 1..29: note = Modified bacterial sequence
EVVAAWDEIDALPNLTLTQWLAFINKLDD

SEQ ID NO: 98 - protein, 29 aa, synthetic construct
  REGION 1..29: note = Modified bacterial sequence
EVIQAWNEIDGLPNLTLSQWLAFINKLDD

SEQ ID NO: 99 - protein, 29 aa, synthetic construct
  REGION 1..29: note = Modified bacterial sequence
ETIEAWDEIDALPNLTITQWLAFINKLDD

SEQ ID NO: 100 - protein, 29 aa, synthetic construct
  REGION 1..29: note = Modified bacterial sequence
EVIDAWNEIDHLPNLTIQQWLAFINKLAD

SEQ ID NO: 101 - protein, 29 aa, synthetic construct
  REGION 1..29: note = Modified bacterial sequence
ETIEAWNEIDALPNLTLDQWLAFINKLED

SEQ ID NO: 102 - protein, 29 aa, synthetic construct
  REGION 1..29: note = Modified bacterial sequence
EHIHAWNEIDELPNLTIEQWLAFINKLAD

SEQ ID NO: 103 - protein, 29 aa, synthetic construct
  REGION 1..29: note = Modified bacterial sequence
EVIDAWDEIDHLPNLTIDQWLAFINKLSD

SEQ ID NO: 104 - protein, 29 aa, synthetic construct
  REGION 1..29: note = Modified bacterial sequence
EVIDANDEIDALPNLTIAQWLAFINKLHD

SEQ ID NO: 105 - protein, 29 aa, synthetic construct
  REGION 1..29: note = Modified bacterial sequence
ETIEAWDEIDKLPNLTIEQWLAFINKLDD

SEQ ID NO: 106 - protein, 29 aa, synthetic construct
  REGION 1..29: note = Modified bacterial sequence
EVLLAWDEIDHLPNLTLEQWLAFINKLDD

SEQ ID NO: 107 - protein, 29 aa, synthetic construct
  REGION 1..29: note = Modified bacterial sequence
EHIDAWNEIDGLPNLTLEQWLAFINKLDD

SEQ ID NO: 108 - protein, 29 aa, synthetic construct
  REGION 1..29: note = Modified bacterial sequence
EVIEAWSEIDALPNLTIDQWLAFINKLAD

SEQ ID NO: 109 - protein, 29 aa, synthetic construct
  REGION 1..29: note = Modified bacterial sequence
EQLNAWAEIDALPNLTIEQWLAFINKLDD

SEQ ID NO: 110 - protein, 29 aa, synthetic construct
  REGION 1..29: note = Modified bacterial sequence
EVIDAWNEIDALPNLTIAQWLAFINKLDD

SEQ ID NO: 111 - protein, 29 aa, synthetic construct
  REGION 1..29: note = Modified bacterial sequence
ETIDAWNEIDQLPNLTIEQWLAFINKLDD

SEQ ID NO: 112 - protein, 29 aa, synthetic construct
  REGION 1..29: note = Modified bacterial sequence
EVIEAWDEIDKLPNLTLAQWLAFINKLDD

SEQ ID NO: 113 - protein, 29 aa, synthetic construct
  REGION 1..29: note = Modified bacterial sequence
EVLYAWAEIDHLPNLTIEQWLAFINKLDD

SEQ ID NO: 114 - protein, 29 aa, synthetic construct
  REGION 1..29: note = Modified bacterial sequence
EQIDAWNEIDRLPNLTIQQWLAFINKLDD

SEQ ID NO: 115 - protein, 29 aa, synthetic construct
  REGION 1..29: note = Modified bacterial sequence
EVLAAWDEIDRLPNLTIEQWLAFINKLDD

SEQ ID NO: 116 - protein, 29 aa, synthetic construct
  REGION 1..29: note = Modified bacterial sequence
EVIEAWDEIDHLPNLTLHQWLAFINKLDD

SEQ ID NO: 117 - protein, 29 aa, synthetic construct
  REGION 1..29: note = Modified bacterial sequence
EVIEAWNEIDKLPNLTLQQWLAFINKLDD

SEQ ID NO: 118 - protein, 29 aa, synthetic construct
  REGION 1..29: note = Modified bacterial sequence
EVIDANDEIDALPNLTIEQWLAFINKLHD

SEQ ID NO: 119 - protein, 29 aa, synthetic construct
  REGION 1..29: note = Modified bacterial sequence
EVIAAWDEIDALPNLTIEQWLAFINKLDD

SEQ ID NO: 120 - protein, 29 aa, synthetic construct
  REGION 1..29: note = Modified bacterial sequence
EVIEAWTEIDQLPNLTLDQWLAFINKLDD

SEQ ID NO: 121 - protein, 29 aa, synthetic construct
  REGION 1..29: note = Modified bacterial sequence
EVINAWNEIDALPNLTLQQWLAFINKLDD

SEQ ID NO: 122 - protein, 29 aa, synthetic construct
  REGION 1..29: note = Modified bacterial sequence
EHIEAWDEIDHLPNLTIDQWLAFINKLAD

SEQ ID NO: 123 - protein, 29 aa, synthetic construct
  REGION 1..29: note = Modified bacterial sequence
EHLEAWREIDALPNLTIEQWLAFINKLDD

SEQ ID NO: 124 - protein, 29 aa, synthetic construct
  REGION 1..29: note = Modified bacterial sequence
EVLDAWNEIDKLPNLTLQQWLAFINKLDD

SEQ ID NO: 125 - protein, 29 aa, synthetic construct
  REGION 1..29: note = Modified bacterial sequence
EVIAAWDEIDHLPNLTIQQWLAFINKLDD

SEQ ID NO: 126 - protein, 29 aa, synthetic construct
  REGION 1..29: note = Modified bacterial sequence
EVIQAWNEIDALPNLTLEQWLAFINKLDD

SEQ ID NO: 127 - protein, 29 aa, synthetic construct
  REGION 1..29: note = Modified bacterial sequence
EVIDAWNEIDHLPNLTIAQWLAFINKLDD

SEQ ID NO: 128 - protein, 29 aa, synthetic construct
  REGION 1..29: note = Modified bacterial sequence
EQLDAWDEIDHLPNLTIDQWLAFINKLSD

SEQ ID NO: 129 - protein, 29 aa, synthetic construct
  REGION 1..29: note = Modified bacterial sequence
EVLNAWDEIDKLPNLTIEQWLAFINKLDD

SEQ ID NO: 130 - protein, 29 aa, synthetic construct
  REGION 1..29: note = Modified bacterial sequence
EVLEAWNEIDHLPNLTIDQWLAFINKLDD

SEQ ID NO: 131 - protein, 29 aa, synthetic construct
  REGION 1..29: note = Modified bacterial sequence
EVLLAWDEIDRLPNLTIDQWLAFINKLAD

SEQ ID NO: 132 - protein, 29 aa, synthetic construct
  REGION 1..29: note = Modified bacterial sequence
EVIAAWNEIDQLPNLTLDQWLAFINKLDD

SEQ ID NO: 133 - protein, 29 aa, synthetic construct
  REGION 1..29: note = Modified bacterial sequence
ETLLAWDEIDALPNLTIEQWLAFINKLDD

SEQ ID NO: 134 - protein, 29 aa, synthetic construct
  REGION 1..29: note = Modified bacterial sequence
EVIDAWNEIDTLPNLTLEQWLAFINKLDD

SEQ ID NO: 135 - protein, 29 aa, synthetic construct
  REGION 1..29: note = Modified bacterial sequence
EVLHAWNEIDHLPNLTLNQWLAFINKLQD

SEQ ID NO: 136 - protein, 29 aa, synthetic construct
  REGION 1..29: note = Modified bacterial sequence
EVIQAWNEIDALPNLTIAQWLAFINKLDD

SEQ ID NO: 137 - protein, 29 aa, synthetic construct
  REGION 1..29: note = Modified bacterial sequence
ETVDAWNEIDALPNLTIEQWLAFINKLDD

SEQ ID NO: 138 - protein, 29 aa, synthetic construct
  REGION 1..29: note = Modified bacterial sequence
EVIQAWDEIDHLPNLTIDQWLAFINKLDD

SEQ ID NO: 139 - protein, 29 aa, synthetic construct
  REGION 1..29: note = Modified bacterial sequence
EVLDAWNEIDQLPNLTIQQWLAFINKLDD

SEQ ID NO: 140 - protein, 29 aa, synthetic construct
  REGION 1..29: note = Modified bacterial sequence
ETIEAWNEIDALPNLTLDQWLAFINKLDD

SEQ ID NO: 141 - protein, 29 aa, synthetic construct
  REGION 1..29: note = Modified bacterial sequence
EVIEAWDEIDALPNLTIDQWLAFINKLDD

SEQ ID NO: 142 - protein, 29 aa, synthetic construct
  REGION 1..29: note = Modified bacterial sequence
EVIEAWNEIDQLPNLTIQQWLAFINKLDD

SEQ ID NO: 143 - protein, 29 aa, synthetic construct
  REGION 1..29: note = Modified bacterial sequence
EVIEAWTEIDHLPNLTIEQWLAFINKLDD

SEQ ID NO: 144 - protein, 29 aa, synthetic construct
  REGION 1..29: note = Modified bacterial sequence
EVIQAWNEIDHLPNLTLQQWLAFINKLED

SEQ ID NO: 145 - protein, 29 aa, synthetic construct
  REGION 1..29: note = Modified bacterial sequence
EVIQANNEIDQLPNLTIEQWLAFINKLHD

SEQ ID NO: 146 - protein, 29 aa, synthetic construct
  REGION 1..29: note = Modified bacterial sequence
EVLHAWSEIDKLPNLTIEQWLAFINKLDD

SEQ ID NO: 147 - protein, 29 aa, synthetic construct
  REGION 1..29: note = Modified bacterial sequence
ETIQAWDEIDKLPNLTLDQWLAFINKLSD

SEQ ID NO: 148 - protein, 29 aa, synthetic construct
  REGION 1..29: note = Modified bacterial sequence
ETLRAWDEIDKLPNLTIQQWLAFINKLAD

SEQ ID NO: 149 - protein, 29 aa, synthetic construct
  REGION 1..29: note = Modified bacterial sequence
EVIDAWNEIDHLPNLTIEQWLAFINKLED

SEQ ID NO: 150 - protein, 29 aa, synthetic construct
  REGION 1..29: note = Modified bacterial sequence
EVIDAWNEIDHLPNLTLQQWLAFINKLAD

SEQ ID NO: 151 - protein, 29 aa, synthetic construct
  REGION 1..29: note = Modified bacterial sequence
ETIDAWNEIDALPNLTLDQWLAFINKLDD

SEQ ID NO: 152 - protein, 29 aa, synthetic construct
  REGION 1..29: note = Modified bacterial sequence
EVIEAWNEIDQLPNLTIEQWLAFINKLDD

SEQ ID NO: 153 - protein, 29 aa, synthetic construct
  REGION 1..29: note = Modified bacterial sequence
EVIRAWDEIDQLPNLTLSQWLAFINKLDD

SEQ ID NO: 154 - protein, 29 aa, synthetic construct
  REGION 1..29: note = Modified bacterial sequence
EVIEAWNEIDRLPNLTIHQWLAFINKLDD

SEQ ID NO: 155 - protein, 29 aa, synthetic construct
  REGION 1..29: note = Modified bacterial sequence
ETIEAWNEIDQLPNLTIEQWLAFINKLDD

SEQ ID NO: 156 - protein, 29 aa, synthetic construct
  REGION 1..29: note = Modified bacterial sequence
EVLTAWAEIDALPNLTLSQWLAFINKLDD

SEQ ID NO: 157 - protein, 29 aa, synthetic construct
  REGION 1..29: note = Modified bacterial sequence
EVIEAWDEIDKLPNLTVDQWLAFINKLDD

SEQ ID NO: 158 - protein, 29 aa, synthetic construct
  REGION 1..29: note = Modified bacterial sequence
EVIDAWNEIDHLPNLTLTQWLAFINKLDD

SEQ ID NO: 159 - protein, 29 aa, synthetic construct
  REGION 1..29: note = Modified bacterial sequence
EVIEAWNEIDQLPNLTLDQWLAFINKLDD

SEQ ID NO: 160 - protein, 29 aa, synthetic construct
  REGION 1..29: note = Modified bacterial sequence
ETLQAWDEIDHLPNLTLNQWLAFINKLDD

SEQ ID NO: 161 - protein, 29 aa, synthetic construct
  REGION 1..29: note = Modified bacterial sequence
EVIDAWNEIDHLPNLTIEQWLAFINKLDD

SEQ ID NO: 162 - protein, 29 aa, synthetic construct
  REGION 1..29: note = Modified bacterial sequence
EVIEAWNEIDLLPNLTLSQWLAFINKLDD

SEQ ID NO: 163 - protein, 29 aa, synthetic construct
  REGION 1..29: note = Modified bacterial sequence
EVIDAWDEIDRLPNLTLKQWLAFINKLDD

SEQ ID NO: 164 - protein, 29 aa, synthetic construct
  REGION 1..29: note = Modified bacterial sequence
ETLHAWDEIDKLPNLTIEQWLAFINKLDD

SEQ ID NO: 165 - protein, 29 aa, synthetic construct
  REGION 1..29: note = Modified bacterial sequence
EVIKAWDEIDHLPNLTLNQWLAFINKLDD

SEQ ID NO: 166 - protein, 29 aa, synthetic construct
  REGION 1..29: note = Modified bacterial sequence
EVIEAWNEIDHLPNLTLAQWLAFINKLDD

SEQ ID NO: 167 - protein, 29 aa, synthetic construct
  REGION 1..29: note = Modified bacterial sequence
EVIQAWNEIDHLPNLTIDQWLAFITKLED

SEQ ID NO: 168 - protein, 29 aa, synthetic construct
  REGION 1..29: note = Modified bacterial sequence
EVIEAWNEIDRLPNLTIKQWLAFINKLDD

SEQ ID NO: 169 - protein, 29 aa, synthetic construct
  REGION 1..29: note = Modified bacterial sequence
EVIEAWNEIDSLPNLTLQQWLAFINKLDD

SEQ ID NO: 170 - protein, 29 aa, synthetic construct
  REGION 1..29: note = Modified bacterial sequence
ETIDAWNEIDKLPNLTIEQWLAFINKLDD

SEQ ID NO: 171 - protein, 29 aa, synthetic construct
  REGION 1..29: note = Modified bacterial sequence
EVLEAWAEIDALPNLTIAQWLAFINKLDD

SEQ ID NO: 172 - protein, 29 aa, synthetic construct
  REGION 1..29: note = Modified bacterial sequence
ETIDAWNEIDRLPNLTIEQWLAFINKLDD

SEQ ID NO: 173 - protein, 29 aa, synthetic construct
  REGION 1..29: note = Modified bacterial sequence
ETLKAWDEIDRLPNLTLEQWLAFINKLDD

SEQ ID NO: 174 - protein, 29 aa, synthetic construct
  REGION 1..29: note = Modified bacterial sequence
ETIAAWNEIDALPNLTLQQWLAFINKLDD

SEQ ID NO: 175 - protein, 29 aa, synthetic construct
  REGION 1..29: note = Modified bacterial sequence
EVLQAWNEIDHLPNLTIQQWLAFINKLDD

SEQ ID NO: 176 - protein, 29 aa, synthetic construct
  REGION 1..29: note = Modified bacterial sequence
EVIEAWSEIDHLPNLTLQQWLAFINKLDD

SEQ ID NO: 177 - protein, 29 aa, synthetic construct
  REGION 1..29: note = Modified bacterial sequence
EVIDAWNEIDGLPNLTIEQWLAFINKLDD

SEQ ID NO: 178 - protein, 29 aa, synthetic construct
  REGION 1..29: note = Modified bacterial sequence
EVIHAWNEIDHLPNLTLNQWLAFINKLED

SEQ ID NO: 179 - protein, 29 aa, synthetic construct
  REGION 1..29: note = Modified bacterial sequence
EVLDAWNEIDSLPNLTLDQWLAFINKLDD

SEQ ID NO: 180 - protein, 29 aa, synthetic construct
  REGION 1..29: note = Modified bacterial sequence
EQIEAWNEIDRLPNLTLEQWLAFINKLDD

SEQ ID NO: 181 - protein, 29 aa, synthetic construct
  REGION 1..29: note = Modified bacterial sequence
EVVDAWNEIDALPNLTLQQWLAFINKLDD

SEQ ID NO: 182 - protein, 29 aa, synthetic construct
  REGION 1..29: note = Modified bacterial sequence
EVIEAWNEIDKLPNLTIEQWLAFINKLDD

SEQ ID NO: 183 - protein, 29 aa, synthetic construct
  REGION 1..29: note = Modified bacterial sequence
EVIEANDEIDRLPNLTIEQWLAFINKLHD

SEQ ID NO: 184 - protein, 29 aa, synthetic construct
  REGION 1..29: note = Modified bacterial sequence
ETLQAWDEIDKLPNLTIEQWLAFINKLDD

SEQ ID NO: 185 - protein, 29 aa, synthetic construct
  REGION 1..29: note = Modified bacterial sequence
EVIEAWDEIDHLPNLTIDQWLAFINKLAD

SEQ ID NO: 186 - protein, 29 aa, synthetic construct
  REGION 1..29: note = Modified bacterial sequence
ETIDAWNEIDHLPNLTLQQWLAFINKLAD

SEQ ID NO: 187 - protein, 29 aa, synthetic construct
  REGION 1..29: note = Modified bacterial sequence
EVIDAWDEIDKLPNLTIEQWLAFINKLDD

SEQ ID NO: 188 - protein, 29 aa, synthetic construct
  REGION 1..29: note = Modified bacterial sequence
EVIEAWNEIDKLPNLTLAQWLAFINKLDD

SEQ ID NO: 189 - protein, 29 aa, synthetic construct
  REGION 1..29: note = Modified bacterial sequence
EVLQAWDEIDKLPNLTIQQWLAFINKLDD

SEQ ID NO: 190 - protein, 29 aa, synthetic construct
  REGION 1..29: note = Modified bacterial sequence
EVIAAWNEIDGLPNLTLQQWLAFINKLDD

SEQ ID NO: 191 - protein, 29 aa, synthetic construct
  REGION 1..29: note = Modified bacterial sequence
ETLNAWNEIDALPNLTLQQWLAFINKLDD

SEQ ID NO: 192 - protein, 29 aa, synthetic construct
  REGION 1..29: note = Modified bacterial sequence
EVLSAWNEIDQLPNLTLEQWLAFINKLDD

SEQ ID NO: 193 - protein, 29 aa, synthetic construct
  REGION 1..29: note = Modified bacterial sequence
ETLEAWDEIDHLPNLTLHQWLAFINKLDD

SEQ ID NO: 194 - protein, 29 aa, synthetic construct
  REGION 1..29: note = Modified bacterial sequence
EQIEAWNEIDHLPNLTLQQWLAFINKLAD

SEQ ID NO: 195 - protein, 29 aa, synthetic construct
  REGION 1..29: note = Modified bacterial sequence
EVVEAWDEIDKLPNLTIEQWLAFINKLDD

SEQ ID NO: 196 - protein, 29 aa, synthetic construct
  REGION 1..29: note = Modified bacterial sequence
EVLEAWNEIDELPNLTIEQWLAFINKLDD

SEQ ID NO: 197 - protein, 29 aa, synthetic construct
  REGION 1..29: note = Modified bacterial sequence
EVIDAWNEIDQLPNLTLQQWLAFINKLDD

SEQ ID NO: 198 - protein, 29 aa, synthetic construct
  REGION 1..29: note = Modified bacterial sequence
ETIDAWDEIDKLPNLTLSQWLAFINKLDD

SEQ ID NO: 199 - protein, 29 aa, synthetic construct
  REGION 1..29: note = Modified bacterial sequence
ETIDAWNEIDQLPNLTLQQWLAFINKLDD

SEQ ID NO: 200 - protein, 29 aa, synthetic construct
  REGION 1..29: note = Modified bacterial sequence
EVIQAWDEIDALPNLTLNQWLAFINKLDD

SEQ ID NO: 201 - protein, 29 aa, synthetic construct
  REGION 1..29: note = Modified bacterial sequence
EVLDAWAEIDQLPNLTLQQWLAFINKLDD

SEQ ID NO: 202 - protein, 29 aa, synthetic construct
  REGION 1..29: note = Modified bacterial sequence
EHIAAWDEIDALPNLTIEQWLAFINKLDD

SEQ ID NO: 203 - protein, 29 aa, synthetic construct
  REGION 1..29: note = Modified bacterial sequence
EVIRAWDEIDALPNLTIEQWLAFINKLDD

SEQ ID NO: 204 - protein, 29 aa, synthetic construct
  REGION 1..29: note = Modified bacterial sequence
EVIDAWDEIDALPNLTIDQWLAFINKLAD

SEQ ID NO: 205 - protein, 29 aa, synthetic construct
  REGION 1..29: note = Modified bacterial sequence
EVIDAWNEIDRLPNLTIQQWLAFINKLDD

SEQ ID NO: 206 - protein, 29 aa, synthetic construct
  REGION 1..29: note = Modified bacterial sequence
EVITAWNEIDHLPNLTLSQWLAFINKLDD

SEQ ID NO: 207 - protein, 29 aa, synthetic construct
  REGION 1..29: note = Modified bacterial sequence
EVIDAWNEIDALPNLTIHQWLAFINKLDD

SEQ ID NO: 208 - protein, 29 aa, synthetic construct
  REGION 1..29: note = Modified bacterial sequence
EQLKAWDEIDKLPNLTIEQWLAFIEKLQD

SEQ ID NO: 209 - protein, 29 aa, synthetic construct
  REGION 1..29: note = Modified bacterial sequence
EHIDAWTEIDHLPNLTIEQWLAFINKLDD

SEQ ID NO: 210 - protein, 29 aa, synthetic construct
  REGION 1..29: note = Modified bacterial sequence
EQLRAWDEIDKLPNLTIEQWLAFINKLQD

SEQ ID NO: 211 - protein, 29 aa, synthetic construct
  REGION 1..29: note = Modified bacterial sequence
EVLEAWREIDSLPNLTIAQWLAFINKLDD

SEQ ID NO: 212 - protein, 29 aa, synthetic construct
  REGION 1..29: note = Modified bacterial sequence
EVIQAWNEIDKLPNLTIEQWLAFINKLDD

SEQ ID NO: 213 - protein, 29 aa, synthetic construct
  REGION 1..29: note = Modified bacterial sequence
EHVEAWNEIDQLPNLTIEQWLAFINKLAD

SEQ ID NO: 214 - protein, 29 aa, synthetic construct
  REGION 1..29: note = Modified bacterial sequence
EVIDAWDEIDALPNLTIDQWLAFINKLSD

SEQ ID NO: 215 - protein, 29 aa, synthetic construct
  REGION 1..29: note = Modified bacterial sequence
EVIEAWNEIDHLPNLTIEQWLAFINKLDD

SEQ ID NO: 216 - protein, 29 aa, synthetic construct
  REGION 1..29: note = Modified bacterial sequence
EVLQAWDEIDKLPNLTIEQWLAFINKLSD

SEQ ID NO: 217 - protein, 29 aa, synthetic construct
  REGION 1..29: note = Modified bacterial sequence
EVIKAWNEIDSLPNLTIEQWLAFINKLDD

SEQ ID NO: 218 - protein, 29 aa, synthetic construct
  REGION 1..29: note = Modified bacterial sequence
EVLEAWHEIDLLPNLTIQQWLAFINKLDD

SEQ ID NO: 219 - protein, 29 aa, synthetic construct
  REGION 1..29: note = Modified bacterial sequence
EVLEAWTEIDRLPNLTLDQWLAFINKLDD

SEQ ID NO: 220 - protein, 29 aa, synthetic construct
  REGION 1..29: note = Modified bacterial sequence
EQLYAWNEIDHLPNLTIEQWLAFIEKLQD

SEQ ID NO: 221 - protein, 29 aa, synthetic construct
  REGION 1..29: note = Modified bacterial sequence
EVLNAWDEIDKLPNLTIKQWLAFINKLDD

SEQ ID NO: 222 - protein, 29 aa, synthetic construct
  REGION 1..29: note = Modified bacterial sequence
EVIRAWDEIDKLPNLTVEQWLAFINKLDD

SEQ ID NO: 223 - protein, 29 aa, synthetic construct
  REGION 1..29: note = Modified bacterial sequence
EVVQAWDEIDQLPNLTLEQWLAFINKLDD

SEQ ID NO: 224 - protein, 29 aa, synthetic construct
  REGION 1..29: note = Modified bacterial sequence
EVIRAWDEIDQLPNLTLEQWLAFINKLDD

SEQ ID NO: 225 - protein, 29 aa, synthetic construct
  REGION 1..29: note = Modified bacterial sequence
ETIDAWNEIDHLPNLTLDQWLAFINKLDD

SEQ ID NO: 226 - protein, 29 aa, synthetic construct
  REGION 1..29: note = Modified bacterial sequence
EVVAAWTEIDLLPNLTLDQWLAFINKLED

SEQ ID NO: 227 - protein, 29 aa, synthetic construct
  REGION 1..29: note = Modified bacterial sequence
EVVAAWDEIDALPNLTIEQWLAFINKLSD

SEQ ID NO: 228 - protein, 29 aa, synthetic construct
  REGION 1..29: note = Modified bacterial sequence
ETLEAWREIDSLPNLTLEQWLAFINKLDD

SEQ ID NO: 229 - protein, 29 aa, synthetic construct
  REGION 1..29: note = Modified bacterial sequence
EVIKAWNEIDHLPNLTLDQWLAFINKLDD

SEQ ID NO: 230 - protein, 29 aa, synthetic construct
  REGION 1..29: note = Modified bacterial sequence
EVLEAWTEIDKLPNLTIDQWLAFINKLDD

SEQ ID NO: 231 - protein, 29 aa, synthetic construct
  REGION 1..29: note = Modified bacterial sequence
ETLEAWDEIDKLPNLTIDQWLAFINKLDD

SEQ ID NO: 232 - protein, 29 aa, synthetic construct
  REGION 1..29: note = Modified bacterial sequence
EVIEAWNEIDKLPNLTIDQWLAFINKLDD

SEQ ID NO: 233 - protein, 29 aa, synthetic construct
  REGION 1..29: note = Modified bacterial sequence
ETIDAWNEIDKLPNLTLEQWLAFINKLDD

SEQ ID NO: 234 - protein, 29 aa, synthetic construct
  REGION 1..29: note = Modified bacterial sequence
ETLDAWDEIDALPNLTIDQWLAFINKLED

SEQ ID NO: 235 - protein, 29 aa, synthetic construct
  REGION 1..29: note = Modified bacterial sequence
EVLSAWNEIDHLPNLTIQQWLAFINKLDD

SEQ ID NO: 236 - protein, 29 aa, synthetic construct
  REGION 1..29: note = Modified bacterial sequence
EVIQANDEIDKLPNLTIEQWLAFIHKLHD

SEQ ID NO: 237 - protein, 29 aa, synthetic construct
  REGION 1..29: note = Modified bacterial sequence
EHLDAWDEIDHLPNLTIQQWLAFINKLAD

SEQ ID NO: 238 - protein, 29 aa, synthetic construct
  REGION 1..29: note = Modified bacterial sequence
EVIQAWNEIDQLPNLTIEQWLAFINKLDD

SEQ ID NO: 239 - protein, 29 aa, synthetic construct
  REGION 1..29: note = Modified bacterial sequence
EVIEAWNEIDYLPNLTIAQWIAFINKLDD

SEQ ID NO: 240 - protein, 29 aa, synthetic construct
  REGION 1..29: note = Modified bacterial sequence
ETIQAWDEIDRLPNLTLQQWLAFINKLDD

SEQ ID NO: 241 - protein, 29 aa, synthetic construct
  REGION 1..29: note = Modified bacterial sequence
ETIQAWDEIDKLPNLTIEQWLAFINKLDD

SEQ ID NO: 242 - protein, 29 aa, synthetic construct
  REGION 1..29: note = Modified bacterial sequence
ETLDAWAEIDHLPNLTIEQWLAFINKLDD

SEQ ID NO: 243 - protein, 29 aa, synthetic construct
  REGION 1..29: note = Modified bacterial sequence
EVIEAWDEIDKLPNLTLNQWLAFINKLDD

SEQ ID NO: 244 - protein, 29 aa, synthetic construct
  REGION 1..29: note = Modified bacterial sequence
EVLDAWNEIDQLPNLTIEQWLAFINKLDD

SEQ ID NO: 245 - protein, 29 aa, synthetic construct
  REGION 1..29: note = Modified bacterial sequence
EVLHAWNEIDHLPNLTIEQWLAFIEKLED

SEQ ID NO: 246 - protein, 29 aa, synthetic construct
  REGION 1..29: note = Modified bacterial sequence
EVIEAWQEIDKLPNLTIDQWLAFINKLDD

SEQ ID NO: 247 - protein, 29 aa, synthetic construct
  REGION 1..29: note = Modified bacterial sequence
EVVDAWNEIDQLPNLTIEQWLAFINKLDD

SEQ ID NO: 248 - protein, 29 aa, synthetic construct
  REGION 1..29: note = Modified bacterial sequence
EQIEAWNEIDALPNLTIEQWLAFINKLAD

SEQ ID NO: 249 - protein, 49 aa, synthetic construct
  REGION 1..49: note = Modified bacterial sequence
KEVLEAWDEIDRLPNLTIEQWLAFINKLDDDPSQSSELLSEAKKLNDSQ

SEQ ID NO: 250 - protein, 49 aa, synthetic construct
  REGION 1..49: note = Modified bacterial sequence
KEVLEAWNEIDRLPNLTIEQWLAFINKLDDDPSQSSELLSEAKKLNDSQ

SEQ ID NO: 251 - protein, 49 aa, synthetic construct
  REGION 1..49: note = Modified bacterial sequence
KEVIEAWNEIDRLPNLTIEQWLAFINKLDDDPSQSSELLSEAKKLNDSQ

SEQ ID NO: 252 - protein, 49 aa, synthetic construct
  REGION 1..49: note = Modified bacterial sequence
KEVLEAWDEIDRLPNLTLDQWLAFINKLDDDPSQSSELLSEAKKLNDSQ

SEQ ID NO: 253 - protein, 49 aa, synthetic construct
  REGION 1..49: note = Modified bacterial sequence
KEVLDAWDEIDALPNLTLEQWLAFINKLDDDPSQSSELLSEAKKLNDSQ

SEQ ID NO: 254 - protein, 49 aa, synthetic construct
  REGION 1..49: note = Modified bacterial sequence
KEVIDAWDEIDRLPNLTLDQWLAFINKLDDDPSQSSELLSEAKKLNDSQ

SEQ ID NO: 255 - protein, 49 aa, synthetic construct
  REGION 1..49: note = Modified bacterial sequence
KETLEAWDEIDRLPNLTIEQWLAFINKLDDDPSQSSELLSEAKKLNDSQ

SEQ ID NO: 256 - protein, 49 aa, synthetic construct
  REGION 1..49: note = Modified bacterial sequence
KEVIDAWNEIDALPNLTLDQWLAFINKLDDDPSQSSELLSEAKKLNDSQ

SEQ ID NO: 257 - protein, 49 aa, synthetic construct
  REGION 1..49: note = Modified bacterial sequence
KEVLDAWDEIDKLPNLTIDQWLAFINKLDDDPSQSSELLSEAKKLNDSQ

SEQ ID NO: 258 - protein, 49 aa, synthetic construct
  REGION 1..49: note = Modified bacterial sequence
KEVLEAWDEIDHLPNLTLDQWLAFINKLDDDPSQSSELLSEAKKLNDSQ

SEQ ID NO: 259 - protein, 49 aa, synthetic construct
  REGION 1..49: note = Modified bacterial sequence
KEVLEAWDEIDALPNLTIEQWLAFINKLDDDPSQSSELLSEAKKLNDSQ

SEQ ID NO: 260 - protein, 49 aa, synthetic construct
  REGION 1..49: note = Modified bacterial sequence
KEVLDAWDEIDKLPNLTLEQWLAFINKLDDDPSQSSELLSEAKKLNDSQ

SEQ ID NO: 261 - protein, 49 aa, synthetic construct
  REGION 1..49: note = Modified bacterial sequence
KETITAWDEIDKLPNLTIEQWLAFIGKLEDDPSQSSELLAEAKKLNDAQ

SEQ ID NO: 262 - protein, 49 aa, synthetic construct
  REGION 1..49: note = Modified bacterial sequence
KESMKAWDEIDRLPNLNINQWVAFIDSLYDDPSQSANLLAEAKKLNDAQ

SEQ ID NO: 263 - protein, 49 aa, synthetic construct
  REGION 1..49: note = Modified bacterial sequence
KESIEAWTEIDHLPNLTIEQWLAFINKLTDDPSQSSELLAEAKKLNDAQ

SEQ ID NO: 264 - protein, 49 aa, synthetic construct
  REGION 1..49: note = Modified bacterial sequence
KEVLDAWHEIDTLPNLTVRQWLAFISKLEDDPSQSSELLAEAKKLNDAQ

SEQ ID NO: 265 - protein, 49 aa, synthetic construct
  REGION 1..49: note = Modified bacterial sequence
KEHIQANEEIDRLPNLTIKQWLAFINKLHDDPSQSSELLAEAKKLNDAQ

SEQ ID NO: 266 - protein, 49 aa, synthetic construct
  REGION 1..49: note = Modified bacterial sequence
KEVLHAWAEIDALPNLTIEQWLAFINKLDDDPSQSSELLSEAKKLNDSQ

SEQ ID NO: 267 - protein, 49 aa, synthetic construct
  REGION 1..49: note = Modified bacterial sequence
KEVLAAWDEIDSLPNLTLQQWLAFINKLDDDPSQSSELLSEAKKLNDSQ

SEQ ID NO: 268 - protein, 49 aa, synthetic construct
  REGION 1..49: note = Modified bacterial sequence
KEVIDAWNEIDALPNLTLEQWLAFINKLDDDPSQSSELLSEAKKLNDSQ

SEQ ID NO: 269 - protein, 49 aa, synthetic construct
  REGION 1..49: note = Modified bacterial sequence
KEVLDAWNEIDALPNLTIDQWLAFINKLSDDPSQSSELLSEAKKLNDSQ

SEQ ID NO: 270 - protein, 49 aa, synthetic construct
  REGION 1..49: note = Modified bacterial sequence
KEVIEAWDEIDGLPNLTIEQWLAFINKLDDDPSQSSELLSEAKKLNDSQ

SEQ ID NO: 271 - protein, 49 aa, synthetic construct
  REGION 1..49: note = Modified bacterial sequence
KEVLEAWDEIDHLPNLTLQQWLAFINKLDDDPSQSSELLSEAKKLNDSQ

SEQ ID NO: 272 - protein, 49 aa, synthetic construct
  REGION 1..49: note = Modified bacterial sequence
KEVIEAWNEIDALPNLTIEQWLAFINKLDDDPSQSSELLSEAKKLNDSQ

SEQ ID NO: 273 - protein, 49 aa, synthetic construct
  REGION 1..49: note = Modified bacterial sequence
KEVIAAWNEIDRLPNLTLTQWLAFINKLDDDPSQSSELLSEAKKLNDSQ

SEQ ID NO: 274 - protein, 49 aa, synthetic construct
  REGION 1..49: note = Modified bacterial sequence
KEVIEAWDEIDALPNLTLQQWLAFINKLDDDPSQSSELLSEAKKLNDSQ

SEQ ID NO: 275 - protein, 49 aa, synthetic construct
  REGION 1..49: note = Modified bacterial sequence
KEVIAAWDEIDKLPNLTIEQWLAFINKLDDDPSQSSELLSEAKKLNDSQ

SEQ ID NO: 276 - protein, 49 aa, synthetic construct
  REGION 1..49: note = Modified bacterial sequence
KEVIAAWDEIDKLPNLTLQQWLAFINKLDDDPSQSSELLSEAKKLNDSQ

SEQ ID NO: 277 - protein, 49 aa, synthetic construct
  REGION 1..49: note = Modified bacterial sequence
KETIAAWDEIDKLPNLTIEQWLAFINKLDDDPSQSSELLSEAKKLNDSQ

SEQ ID NO: 278 - protein, 49 aa, synthetic construct
  REGION 1..49: note = Modified bacterial sequence
KETIEAWNEIDRLPNLTIEQWLAFINKLDDDPSQSSELLSEAKKLNDSQ

SEQ ID NO: 279 - protein, 49 aa, synthetic construct
  REGION 1..49: note = Modified bacterial sequence
KEVLEAWREIDALPNLTIQQWLAFINKLDDDPSQSSELLSEAKKLNDSQ

SEQ ID NO: 280 - protein, 49 aa, synthetic construct
  REGION 1..49: note = Modified bacterial sequence
KEVIEAWDEIDQLPNLTIEQWLAFINKLDDDPSQSSELLSEAKKLNDSQ

SEQ ID NO: 281 - protein, 49 aa, synthetic construct
  REGION 1..49: note = Modified bacterial sequence
KEVLRAWDEIDHLPNLTLEQWLAFINKLDDDPSQSSELLSEAKKLNDSQ

SEQ ID NO: 282 - protein, 49 aa, synthetic construct
  REGION 1..49: note = Modified bacterial sequence
KEVLEAWDEIDRLPNLTLNQWLAFINKLDDDPSQSSELLSEAKKLNDSQ

SEQ ID NO: 283 - protein, 49 aa, synthetic construct
  REGION 1..49: note = Modified bacterial sequence
KEVLDAWNEIDHLPNLTIEQWLAFINKLDDDPSQSSELLSEAKKLNDSQ

SEQ ID NO: 284 - protein, 49 aa, synthetic construct
  REGION 1..49: note = Modified bacterial sequence
KEVIDAWNEIDKLPNLTIEQWLAFINKLDDDPSQSSELLSEAKKLNDSQ

SEQ ID NO: 285 - protein, 49 aa, synthetic construct
  REGION 1..49: note = Modified bacterial sequence
KETLEAWDEIDQLPNLTLQQWLAFINKLDDDPSQSSELLSEAKKLNDSQ

SEQ ID NO: 286 - protein, 49 aa, synthetic construct
  REGION 1..49: note = Modified bacterial sequence
KEVIEAWNEIDALPNLTLDQWLAFINKLDDDPSQSSELLSEAKKLNDSQ

SEQ ID NO: 287 - protein, 49 aa, synthetic construct
  REGION 1..49: note = Modified bacterial sequence
KEVIDAWNEIDRLPNLTLQQWLAFINKLDDDPSQSSELLSEAKKLNDSQ

SEQ ID NO: 288 - protein, 49 aa, synthetic construct
  REGION 1..49: note = Modified bacterial sequence
KEVIDAWNEIDQLPNLTLEQWLAFINKLDDDPSQSSELLSEAKKLNDSQ

SEQ ID NO: 289 - protein, 49 aa, synthetic construct
  REGION 1..49: note = Modified bacterial sequence
KETIAAWDEIDHLPNLTLEQWLAFINKLDDDPSQSSELLSEAKKLNDSQ

SEQ ID NO: 290 - protein, 49 aa, synthetic construct
  REGION 1..49: note = Modified bacterial sequence
KEVLQAWDEIDHLPNLTIQQWLAFINKLSDDPSQSSELLSEAKKLNDSQ

SEQ ID NO: 291 - protein, 49 aa, synthetic construct
  REGION 1..49: note = Modified bacterial sequence
KETLHAWAEIDRLPNLTIEQWLAFINKLDDDPSQSSELLSEAKKLNDSQ

SEQ ID NO: 292 - protein, 49 aa, synthetic construct
  REGION 1..49: note = Modified bacterial sequence
KEVLEAWNEIDHLPNLTLAQWLAFINKLDDDPSQSSELLSEAKKLNDSQ

SEQ ID NO: 293 - protein, 49 aa, synthetic construct
  REGION 1..49: note = Modified bacterial sequence
KEVIEAWDEIDKLPNLTIAQWLAFINKLDDDPSQSSELLSEAKKLNDSQ

SEQ ID NO: 294 - protein, 49 aa, synthetic construct
  REGION 1..49: note = Modified bacterial sequence
KEVLDAWDEIDHLPNLTLQQWLAFINKLDDDPSQSSELLSEAKKLNDSQ

SEQ ID NO: 295 - protein, 49 aa, synthetic construct
  REGION 1..49: note = Modified bacterial sequence
KETIEAWNEIDKLPNLTLTQWLAFINKLDDDPSQSSELLSEAKKLNDSQ

SEQ ID NO: 296 - protein, 49 aa, synthetic construct
  REGION 1..49: note = Modified bacterial sequence
KEVLEAWNEIDLLPNLTIEQWLAFINKLDDDPSQSSELLSEAKKLNDSQ

SEQ ID NO: 297 - protein, 49 aa, synthetic construct
  REGION 1..49: note = Modified bacterial sequence
KEVIEAWDEIDHLPNLTIDQWLAFINKLDDDPSQSSELLSEAKKLNDSQ

SEQ ID NO: 298 - protein, 49 aa, synthetic construct
  REGION 1..49: note = Modified bacterial sequence
KEVISAWNEIDALPNLTLQQWLAFINKLDDDPSQSSELLSEAKKLNDSQ

SEQ ID NO: 299 - protein, 49 aa, synthetic construct
  REGION 1..49: note = Modified bacterial sequence
KEVIAAWNEIDKLPNLTLEQWLAFINKLDDDPSQSSELLSEAKKLNDSQ

SEQ ID NO: 300 - protein, 49 aa, synthetic construct
  REGION 1..49: note = Modified bacterial sequence
KETIEAWNEIDSLPNLTLDQWLAFINKLDDDPSQSSELLSEAKKLNDSQ

SEQ ID NO: 301 - protein, 49 aa, synthetic construct
  REGION 1..49: note = Modified bacterial sequence
KEVLDAWNEIDQLPNLTLQQWLAFINKLDDDPSQSSELLSEAKKLNDSQ

SEQ ID NO: 302 - protein, 49 aa, synthetic construct
  REGION 1..49: note = Modified bacterial sequence
KEVLAAWNEIDHLPNLTIEQWLAFINKLDDDPSQSSELLSEAKKLNDSQ

SEQ ID NO: 303 - protein, 49 aa, synthetic construct
  REGION 1..49: note = Modified bacterial sequence
KEVLEAWDEIDHLPNLTITQWLAFINKLDDDPSQSSELLSEAKKLNDSQ

SEQ ID NO: 304 - protein, 49 aa, synthetic construct
  REGION 1..49: note = Modified bacterial sequence
KETIDAWNEIDHLPNLTIEQWLAFINKLDDDPSQSSELLSEAKKLNDSQ

SEQ ID NO: 305 - protein, 49 aa, synthetic construct
  REGION 1..49: note = Modified bacterial sequence
KEVIEAWNEIDHLPNLTIQQWLAFINKLDDDPSQSSELLSEAKKLNDSQ

SEQ ID NO: 306 - protein, 49 aa, synthetic construct
  REGION 1..49: note = Modified bacterial sequence
KEVIQAWNEIDALPNLTISQWLAFINKLDDDPSQSSELLSEAKKLNDSQ

SEQ ID NO: 307 - protein, 49 aa, synthetic construct
  REGION 1..49: note = Modified bacterial sequence
KEVIAAWDEIDSLPNLTIEQWLAFINKLDDDPSQSSELLSEAKKLNDSQ

SEQ ID NO: 308 - protein, 49 aa, synthetic construct
  REGION 1..49: note = Modified bacterial sequence
KEHIEAWNEIDALPNLTIEQWLAFINKLQDDPSQSSELLSEAKKLNDSQ

SEQ ID NO: 309 - protein, 49 aa, synthetic construct
  REGION 1..49: note = Modified bacterial sequence
KEVLEAWNEIDKLPNLTLDQWLAFINKLDDDPSQSSELLSEAKKLNDSQ

SEQ ID NO: 310 - protein, 49 aa, synthetic construct
  REGION 1..49: note = Modified bacterial sequence
KEVIDAWNEIDHLPNLTIEQWLAFINKLADDPSQSSELLSEAKKLNDSQ

SEQ ID NO: 311 - protein, 49 aa, synthetic construct
  REGION 1..49: note = Modified bacterial sequence
KETIDAWDEIDKLPNLTIEQWLAFINKLDDDPSQSSELLSEAKKLNDSQ

SEQ ID NO: 312 - protein, 49 aa, synthetic construct
  REGION 1..49: note = Modified bacterial sequence
KEVIAAWDEIDLLPNLTLQQWLAFINKLADDPSQSSELLSEAKKLNDSQ

SEQ ID NO: 313 - protein, 49 aa, synthetic construct
  REGION 1..49: note = Modified bacterial sequence
KEVIHAWDEIDKLPNLTIEQWLAFINKLDDDPSQSSELLSEAKKLNDSQ

SEQ ID NO: 314 - protein, 49 aa, synthetic construct
  REGION 1..49: note = Modified bacterial sequence
KEVIAAWNEIDHLPNLTLEQWLAFINKLDDDPSQSSELLSEAKKLNDSQ

SEQ ID NO: 315 - protein, 49 aa, synthetic construct
  REGION 1..49: note = Modified bacterial sequence
KETLDAWNEIDKLPNLTLSQWLAFINKLDDDPSQSSELLSEAKKLNDSQ

SEQ ID NO: 316 - protein, 49 aa, synthetic construct
  REGION 1..49: note = Modified bacterial sequence
KEVLEAWNEIDALPNLTLEQWLAFINKLDDDPSQSSELLSEAKKLNDSQ

SEQ ID NO: 317 - protein, 49 aa, synthetic construct
  REGION 1..49: note = Modified bacterial sequence
KEVIQAWDEIDHLPNLTISQWLAFINKLDDDPSQSSELLSEAKKLNDSQ

SEQ ID NO: 318 - protein, 49 aa, synthetic construct
  REGION 1..49: note = Modified bacterial sequence
KEVLQAWDEIDSLPNLTIEQWLAFINKLDDDPSQSSELLSEAKKLNDSQ

SEQ ID NO: 319 - protein, 49 aa, synthetic construct
  REGION 1..49: note = Modified bacterial sequence
KETLEAWDEIDHLPNLTIAQWLAFINKLDDDPSQSSELLSEAKKLNDSQ

SEQ ID NO: 320 - protein, 49 aa, synthetic construct
  REGION 1..49: note = Modified bacterial sequence
KETIDAWNEIDRLPNLTISQWLAFINKLDDDPSQSSELLSEAKKLNDSQ

SEQ ID NO: 321 - protein, 49 aa, synthetic construct
  REGION 1..49: note = Modified bacterial sequence
KEVLDAWHEIDHLPNLTIQQWLAFINKLDDDPSQSSELLSEAKKLNDSQ

SEQ ID NO: 322 - protein, 49 aa, synthetic construct
  REGION 1..49: note = Modified bacterial sequence
KEQIRAWDEIDKLPNLTIEQWLAFINKLADDPSQSSELLSEAKKLNDSQ

SEQ ID NO: 323 - protein, 49 aa, synthetic construct
  REGION 1..49: note = Modified bacterial sequence
KETLYAWNEIDKLPNLTIEQWLAFIEKLQDDPSQSSELLSEAKKLNDSQ

SEQ ID NO: 324 - protein, 49 aa, synthetic construct
  REGION 1..49: note = Modified bacterial sequence
KEVIEAWNEIDALPNLTIDQWLAFINKLDDDPSQSSELLSEAKKLNDSQ

SEQ ID NO: 325 - protein, 49 aa, synthetic construct
  REGION 1..49: note = Modified bacterial sequence
KEVLEAWNEIDHLPNLTIQQWLAFINKLDDDPSQSSELLSEAKKLNDSQ

SEQ ID NO: 326 - protein, 49 aa, synthetic construct
  REGION 1..49: note = Modified bacterial sequence
KETIEAWDEIDALPNLTIEQWLAFINKLDDDPSQSSELLSEAKKLNDSQ

SEQ ID NO: 327 - protein, 49 aa, synthetic construct
  REGION 1..49: note = Modified bacterial sequence
KEVIEAWNEIDHLPNLTLQQWLAFINKLDDDPSQSSELLSEAKKLNDSQ

SEQ ID NO: 328 - protein, 49 aa, synthetic construct
  REGION 1..49: note = Modified bacterial sequence
KEVIEAWNEIDKLPNLTIQQWLAFINKLDDDPSQSSELLSEAKKLNDSQ

SEQ ID NO: 329 - protein, 49 aa, synthetic construct
  REGION 1..49: note = Modified bacterial sequence
KETLDAWAEIDHLPNLTLDQWLAFINKLDDDPSQSSELLSEAKKLNDSQ

SEQ ID NO: 330 - protein, 49 aa, synthetic construct
  REGION 1..49: note = Modified bacterial sequence
KEHIDAWNEIDALPNLTLSQWLAFINKLDDDPSQSSELLSEAKKLNDSQ

SEQ ID NO: 331 - protein, 49 aa, synthetic construct
  REGION 1..49: note = Modified bacterial sequence
KEVLDAWNEIDKLPNLTIAQWLAFINKLDDDPSQSSELLSEAKKLNDSQ

SEQ ID NO: 332 - protein, 49 aa, synthetic construct
  REGION 1..49: note = Modified bacterial sequence
KEVIEAWTEIDYLPNLTLQQWLAFINKLDDDPSQSSELLSEAKKLNDSQ

SEQ ID NO: 333 - protein, 49 aa, synthetic construct
  REGION 1..49: note = Modified bacterial sequence
KETIEAWNEIDHLPNLTIAQWLAFINKLDDDPSQSSELLSEAKKLNDSQ

SEQ ID NO: 334 - protein, 49 aa, synthetic construct
  REGION 1..49: note = Modified bacterial sequence
KEVIQAWNEIDKLPNLTLEQWLAFINKLDDDPSQSSELLSEAKKLNDSQ

SEQ ID NO: 335 - protein, 49 aa, synthetic construct
  REGION 1..49: note = Modified bacterial sequence
KEVIEAWDEIDHLPNLTIEQWLAFINKLDDDPSQSSELLSEAKKLNDSQ

SEQ ID NO: 336 - protein, 49 aa, synthetic construct
  REGION 1..49: note = Modified bacterial sequence
KETIDAWNEIDLLPNLTIEQWLAFINKLDDDPSQSSELLSEAKKLNDSQ

SEQ ID NO: 337 - protein, 49 aa, synthetic construct
  REGION 1..49: note = Modified bacterial sequence
KEHIDAWNEIDKLPNLTLDQWLAFINKLDDDPSQSSELLSEAKKLNDSQ

SEQ ID NO: 338 - protein, 49 aa, synthetic construct
  REGION 1..49: note = Modified bacterial sequence
KEVVAAWNEIDALPNLTIEQWLAFINKLNDDPSQSSELLSEAKKLNDSQ

SEQ ID NO: 339 - protein, 49 aa, synthetic construct
  REGION 1..49: note = Modified bacterial sequence
KEVIEAWNEIDALPNLTLAQWLAFINKLDDDPSQSSELLSEAKKLNDSQ

SEQ ID NO: 340 - protein, 49 aa, synthetic construct
  REGION 1..49: note = Modified bacterial sequence
KEVLQAWDEIDRLPNLTLDQWLAFINKLDDDPSQSSELLSEAKKLNDSQ

SEQ ID NO: 341 - protein, 49 aa, synthetic construct
  REGION 1..49: note = Modified bacterial sequence
KEVIDAWDEIDHLPNLTIEQWLAFINKLSDDPSQSSELLSEAKKLNDSQ

SEQ ID NO: 342 - protein, 49 aa, synthetic construct
  REGION 1..49: note = Modified bacterial sequence
KEVVEAWNEIDQLPNLTIEQWLAFINKLDDDPSQSSELLSEAKKLNDSQ

SEQ ID NO: 343 - protein, 49 aa, synthetic construct
  REGION 1..49: note = Modified bacterial sequence
KEVIQAWNEIDALPNLTIEQWLAFINKLDDDPSQSSELLSEAKKLNDSQ

SEQ ID NO: 344 - protein, 49 aa, synthetic construct
  REGION 1..49: note = Modified bacterial sequence
KEVIQAWDEIDKLPNLTIDQWLAFINKLADDPSQSSELLSEAKKLNDSQ

SEQ ID NO: 345 - protein, 49 aa, synthetic construct
  REGION 1..49: note = Modified bacterial sequence
KEVVAAWDEIDALPNLTLTQWLAFINKLDDDPSQSSELLSEAKKLNDSQ

SEQ ID NO: 346 - protein, 49 aa, synthetic construct
  REGION 1..49: note = Modified bacterial sequence
KEVIQAWNEIDGLPNLTLSQWLAFINKLDDDPSQSSELLSEAKKLNDSQ

SEQ ID NO: 347 - protein, 49 aa, synthetic construct
  REGION 1..49: note = Modified bacterial sequence
KETIEAWDEIDALPNLTITQWLAFINKLDDDPSQSSELLSEAKKLNDSQ

SEQ ID NO: 348 - protein, 49 aa, synthetic construct
  REGION 1..49: note = Modified bacterial sequence
KEVIDAWNEIDHLPNLTIQQWLAFINKLADDPSQSSELLSEAKKLNDSQ

SEQ ID NO: 349 - protein, 49 aa, synthetic construct
  REGION 1..49: note = Modified bacterial sequence
KETIEAWNEIDALPNLTLDQWLAFINKLEDDPSQSSELLSEAKKLNDSQ

SEQ ID NO: 350 - protein, 49 aa, synthetic construct
  REGION 1..49: note = Modified bacterial sequence
KEHIHAWNEIDELPNLTIEQWLAFINKLADDPSQSSELLSEAKKLNDSQ

SEQ ID NO: 351 - protein, 49 aa, synthetic construct
  REGION 1..49: note = Modified bacterial sequence
KEVIDAWDEIDHLPNLTIDQWLAFINKLSDDPSQSSELLSEAKKLNDSQ

SEQ ID NO: 352 - protein, 49 aa, synthetic construct
  REGION 1..49: note = Modified bacterial sequence
KEVIDANDEIDALPNLTIAQWLAFINKLHDDPSQSSELLSEAKKLNDSQ

SEQ ID NO: 353 - protein, 49 aa, synthetic construct
  REGION 1..49: note = Modified bacterial sequence
KETIEAWDEIDKLPNLTIEQWLAFINKLDDDPSQSSELLSEAKKLNDSQ

SEQ ID NO: 354 - protein, 49 aa, synthetic construct
  REGION 1..49: note = Modified bacterial sequence
KEVLLAWDEIDHLPNLTLEQWLAFINKLDDDPSQSSELLSEAKKLNDSQ

SEQ ID NO: 355 - protein, 49 aa, synthetic construct
  REGION 1..49: note = Modified bacterial sequence
KEHIDAWNEIDGLPNLTLEQWLAFINKLDDDPSQSSELLSEAKKLNDSQ

SEQ ID NO: 356 - protein, 49 aa, synthetic construct
  REGION 1..49: note = Modified bacterial sequence
KEVIEAWSEIDALPNLTIDQWLAFINKLADDPSQSSELLSEAKKLNDSQ

SEQ ID NO: 357 - protein, 49 aa, synthetic construct
  REGION 1..49: note = Modified bacterial sequence
KEQLNAWAEIDALPNLTIEQWLAFINKLDDDPSQSSELLSEAKKLNDSQ

SEQ ID NO: 358 - protein, 49 aa, synthetic construct
  REGION 1..49: note = Modified bacterial sequence
KEVIDAWNEIDALPNLTIAQWLAFINKLDDDPSQSSELLSEAKKLNDSQ

SEQ ID NO: 359 - protein, 49 aa, synthetic construct
  REGION 1..49: note = Modified bacterial sequence
KETIDAWNEIDQLPNLTIEQWLAFINKLDDDPSQSSELLSEAKKLNDSQ

SEQ ID NO: 360 - protein, 49 aa, synthetic construct
  REGION 1..49: note = Modified bacterial sequence
KEVIEAWDEIDKLPNLTLAQWLAFINKLDDDPSQSSELLSEAKKLNDSQ

SEQ ID NO: 361 - protein, 49 aa, synthetic construct
  REGION 1..49: note = Modified bacterial sequence
KEVLYAWAEIDHLPNLTIEQWLAFINKLDDDPSQSSELLSEAKKLNDSQ

SEQ ID NO: 362 - protein, 49 aa, synthetic construct
  REGION 1..49: note = Modified bacterial sequence
KEQIDAWNEIDRLPNLTIQQWLAFINKLDDDPSQSSELLSEAKKLNDSQ

SEQ ID NO: 363 - protein, 49 aa, synthetic construct
  REGION 1..49: note = Modified bacterial sequence
KEVLAAWDEIDRLPNLTIEQWLAFINKLDDDPSQSSELLSEAKKLNDSQ

SEQ ID NO: 364 - protein, 49 aa, synthetic construct
  REGION 1..49: note = Modified bacterial sequence
KEVIEAWDEIDHLPNLTLHQWLAFINKLDDDPSQSSELLSEAKKLNDSQ

SEQ ID NO: 365 - protein, 49 aa, synthetic construct
  REGION 1..49: note = Modified bacterial sequence
KEVIEAWNEIDKLPNLTLQQWLAFINKLDDDPSQSSELLSEAKKLNDSQ

SEQ ID NO: 366 - protein, 49 aa, synthetic construct
  REGION 1..49: note = Modified bacterial sequence
KEVIDANDEIDALPNLTIEQWLAFINKLHDDPSQSSELLSEAKKLNDSQ

SEQ ID NO: 367 - protein, 49 aa, synthetic construct
  REGION 1..49: note = Modified bacterial sequence
KEVIAAWDEIDALPNLTIEQWLAFINKLDDDPSQSSELLSEAKKLNDSQ

SEQ ID NO: 368 - protein, 49 aa, synthetic construct
  REGION 1..49: note = Modified bacterial sequence
KEVIEAWTEIDQLPNLTLDQWLAFINKLDDDPSQSSELLSEAKKLNDSQ

SEQ ID NO: 369 - protein, 49 aa, synthetic construct
  REGION 1..49: note = Modified bacterial sequence
KEVINAWNEIDALPNLTLQQWLAFINKLDDDPSQSSELLSEAKKLNDSQ

SEQ ID NO: 370 - protein, 49 aa, synthetic construct
  REGION 1..49: note = Modified bacterial sequence
KEHIEAWDEIDHLPNLTIDQWLAFINKLADDPSQSSELLSEAKKLNDSQ

SEQ ID NO: 371 - protein, 49 aa, synthetic construct
  REGION 1..49: note = Modified bacterial sequence
KEHLEAWREIDALPNLTIEQWLAFINKLDDDPSQSSELLSEAKKLNDSQ

SEQ ID NO: 372 - protein, 49 aa, synthetic construct
  REGION 1..49: note = Modified bacterial sequence
KEVLDAWNEIDKLPNLTLQQWLAFINKLDDDPSQSSELLSEAKKLNDSQ

SEQ ID NO: 373 - protein, 49 aa, synthetic construct
  REGION 1..49: note = Modified bacterial sequence
KEVIAAWDEIDHLPNLTIQQWLAFINKLDDDPSQSSELLSEAKKLNDSQ

SEQ ID NO: 374 - protein, 49 aa, synthetic construct
  REGION 1..49: note = Modified bacterial sequence
KEVIQAWNEIDALPNLTLEQWLAFINKLDDDPSQSSELLSEAKKLNDSQ

SEQ ID NO: 375 - protein, 49 aa, synthetic construct
  REGION 1..49: note = Modified bacterial sequence
KEVIDAWNEIDHLPNLTIAQWLAFINKLDDDPSQSSELLSEAKKLNDSQ

SEQ ID NO: 376 - protein, 49 aa, synthetic construct
  REGION 1..49: note = Modified bacterial sequence
KEQLDAWDEIDHLPNLTIDQWLAFINKLSDDPSQSSELLSEAKKLNDSQ

SEQ ID NO: 377 - protein, 49 aa, synthetic construct
  REGION 1..49: note = Modified bacterial sequence
KEVLNAWDEIDKLPNLTIEQWLAFINKLDDDPSQSSELLSEAKKLNDSQ

SEQ ID NO: 378 - protein, 49 aa, synthetic construct
  REGION 1..49: note = Modified bacterial sequence
KEVLEAWNEIDHLPNLTIDQWLAFINKLDDDPSQSSELLSEAKKLNDSQ

SEQ ID NO: 379 - protein, 49 aa, synthetic construct
  REGION 1..49: note = Modified bacterial sequence
KEVLLAWDEIDRLPNLTIDQWLAFINKLADDPSQSSELLSEAKKLNDSQ

SEQ ID NO: 380 - protein, 49 aa, synthetic construct
  REGION 1..49: note = Modified bacterial sequence
KEVIAAWNEIDQLPNLTLDQWLAFINKLDDDPSQSSELLSEAKKLNDSQ

SEQ ID NO: 381 - protein, 49 aa, synthetic construct
  REGION 1..49: note = Modified bacterial sequence
KETLLAWDEIDALPNLTIEQWLAFINKLDDDPSQSSELLSEAKKLNDSQ

SEQ ID NO: 382 - protein, 49 aa, synthetic construct
  REGION 1..49: note = Modified bacterial sequence
KEVIDAWNEIDTLPNLTLEQWLAFINKLDDDPSQSSELLSEAKKLNDSQ

SEQ ID NO: 383 - protein, 49 aa, synthetic construct
  REGION 1..49: note = Modified bacterial sequence
KEVLHAWNEIDHLPNLTLNQWLAFINKLQDDPSQSSELLSEAKKLNDSQ

SEQ ID NO: 384 - protein, 49 aa, synthetic construct
  REGION 1..49: note = Modified bacterial sequence
KEVIQAWNEIDALPNLTIAQWLAFINKLDDDPSQSSELLSEAKKLNDSQ

SEQ ID NO: 385 - protein, 49 aa, synthetic construct
  REGION 1..49: note = Modified bacterial sequence
KETVDAWNEIDALPNLTIEQWLAFINKLDDDPSQSSELLSEAKKLNDSQ

SEQ ID NO: 386 - protein, 49 aa, synthetic construct
  REGION 1..49: note = Modified bacterial sequence
KEVIQAWDEIDHLPNLTIDQWLAFINKLDDDPSQSSELLSEAKKLNDSQ

SEQ ID NO: 387 - protein, 49 aa, synthetic construct
  REGION 1..49: note = Modified bacterial sequence
KEVLDAWNEIDQLPNLTIQQWLAFINKLDDDPSQSSELLSEAKKLNDSQ

SEQ ID NO: 388 - protein, 49 aa, synthetic construct
  REGION 1..49: note = Modified bacterial sequence
KETIEAWNEIDALPNLTLDQWLAFINKLDDDPSQSSELLSEAKKLNDSQ

SEQ ID NO: 389 - protein, 49 aa, synthetic construct
  REGION 1..49: note = Modified bacterial sequence
KEVIEAWDEIDALPNLTIDQWLAFINKLDDDPSQSSELLSEAKKLNDSQ

SEQ ID NO: 390 - protein, 49 aa, synthetic construct
  REGION 1..49: note = Modified bacterial sequence
KEVIEAWNEIDQLPNLTIQQWLAFINKLDDDPSQSSELLSEAKKLNDSQ

SEQ ID NO: 391 - protein, 49 aa, synthetic construct
  REGION 1..49: note = Modified bacterial sequence
KEVIEAWTEIDHLPNLTIEQWLAFINKLDDDPSQSSELLSEAKKLNDSQ

SEQ ID NO: 392 - protein, 49 aa, synthetic construct
  REGION 1..49: note = Modified bacterial sequence
KEVIQAWNEIDHLPNLTLQQWLAFINKLEDDPSQSSELLSEAKKLNDSQ

SEQ ID NO: 393 - protein, 49 aa, synthetic construct
  REGION 1..49: note = Modified bacterial sequence
KEVIQANNEIDQLPNLTIEQWLAFINKLHDDPSQSSELLSEAKKLNDSQ

SEQ ID NO: 394 - protein, 49 aa, synthetic construct
  REGION 1..49: note = Modified bacterial sequence
KEVLHAWSEIDKLPNLTIEQWLAFINKLDDDPSQSSELLSEAKKLNDSQ

SEQ ID NO: 395 - protein, 49 aa, synthetic construct
  REGION 1..49: note = Modified bacterial sequence
KETIQAWDEIDKLPNLTLDQWLAFINKLSDDPSQSSELLSEAKKLNDSQ

SEQ ID NO: 396 - protein, 49 aa, synthetic construct
  REGION 1..49: note = Modified bacterial sequence
KETLRAWDEIDKLPNLTIQQWLAFINKLADDPSQSSELLSEAKKLNDSQ

SEQ ID NO: 397 - protein, 49 aa, synthetic construct
  REGION 1..49: note = Modified bacterial sequence
KEVIDAWNEIDHLPNLTIEQWLAFINKLEDDPSQSSELLSEAKKLNDSQ

SEQ ID NO: 398 - protein, 49 aa, synthetic construct
  REGION 1..49: note = Modified bacterial sequence
KEVIDAWNEIDHLPNLTLQQWLAFINKLADDPSQSSELLSEAKKLNDSQ

SEQ ID NO: 399 - protein, 49 aa, synthetic construct
  REGION 1..49: note = Modified bacterial sequence
KETIDAWNEIDALPNLTLDQWLAFINKLDDDPSQSSELLSEAKKLNDSQ

SEQ ID NO: 400 - protein, 49 aa, synthetic construct
  REGION 1..49: note = Modified bacterial sequence
KEVIEAWNEIDQLPNLTIEQWLAFINKLDDDPSQSSELLSEAKKLNDSQ

SEQ ID NO: 401 - protein, 49 aa, synthetic construct
  REGION 1..49: note = Modified bacterial sequence
KEVIRAWDEIDQLPNLTLSQWLAFINKLDDDPSQSSELLSEAKKLNDSQ

SEQ ID NO: 402 - protein, 49 aa, synthetic construct
  REGION 1..49: note = Modified bacterial sequence
KEVIEAWNEIDRLPNLTIHQWLAFINKLDDDPSQSSELLSEAKKLNDSQ

SEQ ID NO: 403 - protein, 49 aa, synthetic construct
  REGION 1..49: note = Modified bacterial sequence
KETIEAWNEIDQLPNLTIEQWLAFINKLDDDPSQSSELLSEAKKLNDSQ

SEQ ID NO: 404 - protein, 49 aa, synthetic construct
  REGION 1..49: note = Modified bacterial sequence
KEVLTAWAEIDALPNLTLSQWLAFINKLDDDPSQSSELLSEAKKLNDSQ

SEQ ID NO: 405 - protein, 49 aa, synthetic construct
  REGION 1..49: note = Modified bacterial sequence
KEVIEAWDEIDKLPNLTVDQWLAFINKLDDDPSQSSELLSEAKKLNDSQ

SEQ ID NO: 406 - protein, 49 aa, synthetic construct
  REGION 1..49: note = Modified bacterial sequence
KEVIDAWNEIDHLPNLTLTQWLAFINKLDDDPSQSSELLSEAKKLNDSQ

SEQ ID NO: 407 - protein, 49 aa, synthetic construct
  REGION 1..49: note = Modified bacterial sequence
KEVIEAWNEIDQLPNLTLDQWLAFINKLDDDPSQSSELLSEAKKLNDSQ

SEQ ID NO: 408 - protein, 49 aa, synthetic construct
  REGION 1..49: note = Modified bacterial sequence
KETLQAWDEIDHLPNLTLNQWLAFINKLDDDPSQSSELLSEAKKLNDSQ

SEQ ID NO: 409 - protein, 49 aa, synthetic construct
  REGION 1..49: note = Modified bacterial sequence
KEVIDAWNEIDHLPNLTIEQWLAFINKLDDDPSQSSELLSEAKKLNDSQ

SEQ ID NO: 410 - protein, 49 aa, synthetic construct
  REGION 1..49: note = Modified bacterial sequence
KEVIEAWNEIDLLPNLTLSQWLAFINKLDDDPSQSSELLSEAKKLNDSQ

SEQ ID NO: 411 - protein, 49 aa, synthetic construct
  REGION 1..49: note = Modified bacterial sequence
KEVIDAWDEIDRLPNLTLKQWLAFINKLDDDPSQSSELLSEAKKLNDSQ

SEQ ID NO: 412 - protein, 49 aa, synthetic construct
  REGION 1..49: note = Modified bacterial sequence
KETLHAWDEIDKLPNLTIEQWLAFINKLDDDPSQSSELLSEAKKLNDSQ

SEQ ID NO: 413 - protein, 49 aa, synthetic construct
  REGION 1..49: note = Modified bacterial sequence
KEVIKAWDEIDHLPNLTLNQWLAFINKLDDDPSQSSELLSEAKKLNDSQ

SEQ ID NO: 414 - protein, 49 aa, synthetic construct
  REGION 1..49: note = Modified bacterial sequence
KEVIEAWNEIDHLPNLTLAQWLAFINKLDDDPSQSSELLSEAKKLNDSQ

SEQ ID NO: 415 - protein, 49 aa, synthetic construct
  REGION 1..49: note = Modified bacterial sequence
KEVIQAWNEIDHLPNLTIDQWLAFITKLEDDPSQSSELLSEAKKLNDSQ

SEQ ID NO: 416 - protein, 49 aa, synthetic construct
  REGION 1..49: note = Modified bacterial sequence
KEVIEAWNEIDRLPNLTIKQWLAFINKLDDDPSQSSELLSEAKKLNDSQ

SEQ ID NO: 417 - protein, 49 aa, synthetic construct
  REGION 1..49: note = Modified bacterial sequence
KEVIEAWNEIDSLPNLTLQQWLAFINKLDDDPSQSSELLSEAKKLNDSQ

SEQ ID NO: 418 - protein, 49 aa, synthetic construct
  REGION 1..49: note = Modified bacterial sequence
KETIDAWNEIDKLPNLTIEQWLAFINKLDDDPSQSSELLSEAKKLNDSQ

SEQ ID NO: 419 - protein, 49 aa, synthetic construct
  REGION 1..49: note = Modified bacterial sequence
KEVLEAWAEIDALPNLTIAQWLAFINKLDDDPSQSSELLSEAKKLNDSQ

SEQ ID NO: 420 - protein, 49 aa, synthetic construct
  REGION 1..49: note = Modified bacterial sequence
KETIDAWNEIDRLPNLTIEQWLAFINKLDDDPSQSSELLSEAKKLNDSQ

SEQ ID NO: 421 - protein, 49 aa, synthetic construct
  REGION 1..49: note = Modified bacterial sequence
KETLKAWDEIDRLPNLTLEQWLAFINKLDDDPSQSSELLSEAKKLNDSQ

SEQ ID NO: 422 - protein, 49 aa, synthetic construct
  REGION 1..49: note = Modified bacterial sequence
KETIAAWNEIDALPNLTLQQWLAFINKLDDDPSQSSELLSEAKKLNDSQ

SEQ ID NO: 423 - protein, 49 aa, synthetic construct
  REGION 1..49: note = Modified bacterial sequence
KEVLQAWNEIDHLPNLTIQQWLAFINKLDDDPSQSSELLSEAKKLNDSQ

SEQ ID NO: 424 - protein, 49 aa, synthetic construct
  REGION 1..49: note = Modified bacterial sequence
KEVIEAWSEIDHLPNLTLQQWLAFINKLDDDPSQSSELLSEAKKLNDSQ

SEQ ID NO: 425 - protein, 49 aa, synthetic construct
  REGION 1..49: note = Modified bacterial sequence
KEVIDAWNEIDGLPNLTIEQWLAFINKLDDDPSQSSELLSEAKKLNDSQ

SEQ ID NO: 426 - protein, 49 aa, synthetic construct
  REGION 1..49: note = Modified bacterial sequence
KEVIHAWNEIDHLPNLTLNQWLAFINKLEDDPSQSSELLSEAKKLNDSQ

SEQ ID NO: 427 - protein, 49 aa, synthetic construct
  REGION 1..49: note = Modified bacterial sequence
KEVLDAWNEIDSLPNLTLDQWLAFINKLDDDPSQSSELLSEAKKLNDSQ

SEQ ID NO: 428 - protein, 49 aa, synthetic construct
  REGION 1..49: note = Modified bacterial sequence
KEQIEAWNEIDRLPNLTLEQWLAFINKLDDDPSQSSELLSEAKKLNDSQ

SEQ ID NO: 429 - protein, 49 aa, synthetic construct
  REGION 1..49: note = Modified bacterial sequence
KEVVDAWNEIDALPNLTLQQWLAFINKLDDDPSQSSELLSEAKKLNDSQ

SEQ ID NO: 430 - protein, 49 aa, synthetic construct
  REGION 1..49: note = Modified bacterial sequence
KEVIEAWNEIDKLPNLTIEQWLAFINKLDDDPSQSSELLSEAKKLNDSQ

SEQ ID NO: 431 - protein, 49 aa, synthetic construct
  REGION 1..49: note = Modified bacterial sequence
KEVIEANDEIDRLPNLTIEQWLAFINKLHDDPSQSSELLSEAKKLNDSQ

SEQ ID NO: 432 - protein, 49 aa, synthetic construct
  REGION 1..49: note = Modified bacterial sequence
KETLQAWDEIDKLPNLTIEQWLAFINKLDDDPSQSSELLSEAKKLNDSQ

SEQ ID NO: 433 - protein, 49 aa, synthetic construct
  REGION 1..49: note = Modified bacterial sequence
KEVIEAWDEIDHLPNLTIDQWLAFINKLADDPSQSSELLSEAKKLNDSQ

SEQ ID NO: 434 - protein, 49 aa, synthetic construct
  REGION 1..49: note = Modified bacterial sequence
KETIDAWNEIDHLPNLTLQQWLAFINKLADDPSQSSELLSEAKKLNDSQ

SEQ ID NO: 435 - protein, 49 aa, synthetic construct
  REGION 1..49: note = Modified bacterial sequence
KEVIDAWDEIDKLPNLTIEQWLAFINKLDDDPSQSSELLSEAKKLNDSQ

SEQ ID NO: 436 - protein, 49 aa, synthetic construct
  REGION 1..49: note = Modified bacterial sequence
KEVIEAWNEIDKLPNLTLAQWLAFINKLDDDPSQSSELLSEAKKLNDSQ

SEQ ID NO: 437 - protein, 49 aa, synthetic construct
  REGION 1..49: note = Modified bacterial sequence
KEVLQAWDEIDKLPNLTIQQWLAFINKLDDDPSQSSELLSEAKKLNDSQ

SEQ ID NO: 438 - protein, 49 aa, synthetic construct
  REGION 1..49: note = Modified bacterial sequence
KEVIAAWNEIDGLPNLTLQQWLAFINKLDDDPSQSSELLSEAKKLNDSQ

SEQ ID NO: 439 - protein, 49 aa, synthetic construct
  REGION 1..49: note = Modified bacterial sequence
KETLNAWNEIDALPNLTLQQWLAFINKLDDDPSQSSELLSEAKKLNDSQ

SEQ ID NO: 440 - protein, 49 aa, synthetic construct
  REGION 1..49: note = Modified bacterial sequence
KEVLSAWNEIDQLPNLTLEQWLAFINKLDDDPSQSSELLSEAKKLNDSQ

SEQ ID NO: 441 - protein, 49 aa, synthetic construct
  REGION 1..49: note = Modified bacterial sequence
KETLEAWDEIDHLPNLTLHQWLAFINKLDDDPSQSSELLSEAKKLNDSQ

SEQ ID NO: 442 - protein, 49 aa, synthetic construct
  REGION 1..49: note = Modified bacterial sequence
KEQIEAWNEIDHLPNLTLQQWLAFINKLADDPSQSSELLSEAKKLNDSQ

SEQ ID NO: 443 - protein, 49 aa, synthetic construct
  REGION 1..49: note = Modified bacterial sequence
KEVVEAWDEIDKLPNLTIEQWLAFINKLDDDPSQSSELLSEAKKLNDSQ

SEQ ID NO: 444 - protein, 49 aa, synthetic construct
  REGION 1..49: note = Modified bacterial sequence
KEVLEAWNEIDELPNLTIEQWLAFINKLDDDPSQSSELLSEAKKLNDSQ

SEQ ID NO: 445 - protein, 49 aa, synthetic construct
  REGION 1..49: note = Modified bacterial sequence
KEVIDAWNEIDQLPNLTLQQWLAFINKLDDDPSQSSELLSEAKKLNDSQ

SEQ ID NO: 446 - protein, 49 aa, synthetic construct
  REGION 1..49: note = Modified bacterial sequence
KETIDAWDEIDKLPNLTLSQWLAFINKLDDDPSQSSELLSEAKKLNDSQ

SEQ ID NO: 447 - protein, 49 aa, synthetic construct
  REGION 1..49: note = Modified bacterial sequence
KETIDAWNEIDQLPNLTLQQWLAFINKLDDDPSQSSELLSEAKKLNDSQ

SEQ ID NO: 448 - protein, 49 aa, synthetic construct
  REGION 1..49: note = Modified bacterial sequence
KEVIQAWDEIDALPNLTLNQWLAFINKLDDDPSQSSELLSEAKKLNDSQ

SEQ ID NO: 449 - protein, 49 aa, synthetic construct
  REGION 1..49: note = Modified bacterial sequence
KEVLDAWAEIDQLPNLTLQQWLAFINKLDDDPSQSSELLSEAKKLNDSQ

SEQ ID NO: 450 - protein, 49 aa, synthetic construct
  REGION 1..49: note = Modified bacterial sequence
KEHIAAWDEIDALPNLTIEQWLAFINKLDDDPSQSSELLSEAKKLNDSQ

SEQ ID NO: 451 - protein, 49 aa, synthetic construct
  REGION 1..49: note = Modified bacterial sequence
KEVIRAWDEIDALPNLTIEQWLAFINKLDDDPSQSSELLSEAKKLNDSQ

SEQ ID NO: 452 - protein, 49 aa, synthetic construct
  REGION 1..49: note = Modified bacterial sequence
KEVIDAWDEIDALPNLTIDQWLAFINKLADDPSQSSELLSEAKKLNDSQ

SEQ ID NO: 453 - protein, 49 aa, synthetic construct
  REGION 1..49: note = Modified bacterial sequence
KEVIDAWNEIDRLPNLTIQQWLAFINKLDDDPSQSSELLSEAKKLNDSQ

SEQ ID NO: 454 - protein, 49 aa, synthetic construct
  REGION 1..49: note = Modified bacterial sequence
KEVITAWNEIDHLPNLTLSQWLAFINKLDDDPSQSSELLSEAKKLNDSQ

SEQ ID NO: 455 - protein, 49 aa, synthetic construct
  REGION 1..49: note = Modified bacterial sequence
KEVIDAWNEIDALPNLTIHQWLAFINKLDDDPSQSSELLSEAKKLNDSQ

SEQ ID NO: 456 - protein, 49 aa, synthetic construct
  REGION 1..49: note = Modified bacterial sequence
KEQLKAWDEIDKLPNLTIEQWLAFIEKLQDDPSQSSELLSEAKKLNDSQ

SEQ ID NO: 457 - protein, 49 aa, synthetic construct
  REGION 1..49: note = Modified bacterial sequence
KEHIDAWTEIDHLPNLTIEQWLAFINKLDDDPSQSSELLSEAKKLNDSQ

SEQ ID NO: 458 - protein, 49 aa, synthetic construct
  REGION 1..49: note = Modified bacterial sequence
KEQLRAWDEIDKLPNLTIEQWLAFINKLQDDPSQSSELLSEAKKLNDSQ

SEQ ID NO: 459 - protein, 49 aa, synthetic construct
  REGION 1..49: note = Modified bacterial sequence
KEVLEAWREIDSLPNLTIAQWLAFINKLDDDPSQSSELLSEAKKLNDSQ

SEQ ID NO: 460 - protein, 49 aa, synthetic construct
  REGION 1..49: note = Modified bacterial sequence
KEVIQAWNEIDKLPNLTIEQWLAFINKLDDDPSQSSELLSEAKKLNDSQ

SEQ ID NO: 461 - protein, 49 aa, synthetic construct
  REGION 1..49: note = Modified bacterial sequence
KEHVEAWNEIDQLPNLTIEQWLAFINKLADDPSQSSELLSEAKKLNDSQ

SEQ ID NO: 462 - protein, 49 aa, synthetic construct
  REGION 1..49: note = Modified bacterial sequence
KEVIDAWDEIDALPNLTIDQWLAFINKLSDDPSQSSELLSEAKKLNDSQ

SEQ ID NO: 463 - protein, 49 aa, synthetic construct
  REGION 1..49: note = Modified bacterial sequence
KEVIEAWNEIDHLPNLTIEQWLAFINKLDDDPSQSSELLSEAKKLNDSQ

SEQ ID NO: 464 - protein, 49 aa, synthetic construct
  REGION 1..49: note = Modified bacterial sequence
KEVLQAWDEIDKLPNLTIEQWLAFINKLSDDPSQSSELLSEAKKLNDSQ

SEQ ID NO: 465 - protein, 49 aa, synthetic construct
  REGION 1..49: note = Modified bacterial sequence
KEVIKAWNEIDSLPNLTIEQWLAFINKLDDDPSQSSELLSEAKKLNDSQ

SEQ ID NO: 466 - protein, 49 aa, synthetic construct
  REGION 1..49: note = Modified bacterial sequence
KEVLEAWHEIDLLPNLTIQQWLAFINKLDDDPSQSSELLSEAKKLNDSQ

SEQ ID NO: 467 - protein, 49 aa, synthetic construct
  REGION 1..49: note = Modified bacterial sequence
KEVLEAWTEIDRLPNLTLDQWLAFINKLDDDPSQSSELLSEAKKLNDSQ

SEQ ID NO: 468 - protein, 49 aa, synthetic construct
  REGION 1..49: note = Modified bacterial sequence
KEQLYAWNEIDHLPNLTIEQWLAFIEKLQDDPSQSSELLSEAKKLNDSQ

SEQ ID NO: 469 - protein, 49 aa, synthetic construct
  REGION 1..49: note = Modified bacterial sequence
KEVLNAWDEIDKLPNLTIKQWLAFINKLDDDPSQSSELLSEAKKLNDSQ

SEQ ID NO: 470 - protein, 49 aa, synthetic construct
  REGION 1..49: note = Modified bacterial sequence
KEVIRAWDEIDKLPNLTVEQWLAFINKLDDDPSQSSELLSEAKKLNDSQ

SEQ ID NO: 471 - protein, 49 aa, synthetic construct
  REGION 1..49: note = Modified bacterial sequence
KEVVQAWDEIDQLPNLTLEQWLAFINKLDDDPSQSSELLSEAKKLNDSQ

SEQ ID NO: 472 - protein, 49 aa, synthetic construct
  REGION 1..49: note = Modified bacterial sequence
KEVIRAWDEIDQLPNLTLEQWLAFINKLDDDPSQSSELLSEAKKLNDSQ

SEQ ID NO: 473 - protein, 49 aa, synthetic construct
  REGION 1..49: note = Modified bacterial sequence
KETIDAWNEIDHLPNLTLDQWLAFINKLDDDPSQSSELLSEAKKLNDSQ

SEQ ID NO: 474 - protein, 49 aa, synthetic construct
  REGION 1..49: note = Modified bacterial sequence
KEVVAAWTEIDLLPNLTLDQWLAFINKLEDDPSQSSELLSEAKKLNDSQ

SEQ ID NO: 475 - protein, 49 aa, synthetic construct
  REGION 1..49: note = Modified bacterial sequence
KEVVAAWDEIDALPNLTIEQWLAFINKLSDDPSQSSELLSEAKKLNDSQ

SEQ ID NO: 476 - protein, 49 aa, synthetic construct
  REGION 1..49: note = Modified bacterial sequence
KETLEAWREIDSLPNLTLEQWLAFINKLDDDPSQSSELLSEAKKLNDSQ

SEQ ID NO: 477 - protein, 49 aa, synthetic construct
  REGION 1..49: note = Modified bacterial sequence
KEVIKAWNEIDHLPNLTLDQWLAFINKLDDDPSQSSELLSEAKKLNDSQ

SEQ ID NO: 478 - protein, 49 aa, synthetic construct
  REGION 1..49: note = Modified bacterial sequence
KEVLEAWTEIDKLPNLTIDQWLAFINKLDDDPSQSSELLSEAKKLNDSQ

SEQ ID NO: 479 - protein, 49 aa, synthetic construct
  REGION 1..49: note = Modified bacterial sequence
KETLEAWDEIDKLPNLTIDQWLAFINKLDDDPSQSSELLSEAKKLNDSQ

SEQ ID NO: 480 - protein, 49 aa, synthetic construct
  REGION 1..49: note = Modified bacterial sequence
KEVIEAWNEIDKLPNLTIDQWLAFINKLDDDPSQSSELLSEAKKLNDSQ

SEQ ID NO: 481 - protein, 49 aa, synthetic construct
  REGION 1..49: note = Modified bacterial sequence
KETIDAWNEIDKLPNLTLEQWLAFINKLDDDPSQSSELLSEAKKLNDSQ

SEQ ID NO: 482 - protein, 49 aa, synthetic construct
  REGION 1..49: note = Modified bacterial sequence
KETLDAWDEIDALPNLTIDQWLAFINKLEDDPSQSSELLSEAKKLNDSQ

SEQ ID NO: 483 - protein, 49 aa, synthetic construct
  REGION 1..49: note = Modified bacterial sequence
KEVLSAWNEIDHLPNLTIQQWLAFINKLDDDPSQSSELLSEAKKLNDSQ

SEQ ID NO: 484 - protein, 49 aa, synthetic construct
  REGION 1..49: note = Modified bacterial sequence
KEVIQANDEIDKLPNLTIEQWLAFIHKLHDDPSQSSELLSEAKKLNDSQ

SEQ ID NO: 485 - protein, 49 aa, synthetic construct
  REGION 1..49: note = Modified bacterial sequence
KEHLDAWDEIDHLPNLTIQQWLAFINKLADDPSQSSELLSEAKKLNDSQ

SEQ ID NO: 486 - protein, 49 aa, synthetic construct
  REGION 1..49: note = Modified bacterial sequence
KEVIQAWNEIDQLPNLTIEQWLAFINKLDDDPSQSSELLSEAKKLNDSQ

SEQ ID NO: 487 - protein, 49 aa, synthetic construct
  REGION 1..49: note = Modified bacterial sequence
KEVIEAWNEIDYLPNLTIAQWIAFINKLDDDPSQSSELLSEAKKLNDSQ

SEQ ID NO: 488 - protein, 49 aa, synthetic construct
  REGION 1..49: note = Modified bacterial sequence
KETIQAWDEIDRLPNLTLQQWLAFINKLDDDPSQSSELLSEAKKLNDSQ

SEQ ID NO: 489 - protein, 49 aa, synthetic construct
  REGION 1..49: note = Modified bacterial sequence
KETIQAWDEIDKLPNLTIEQWLAFINKLDDDPSQSSELLSEAKKLNDSQ

SEQ ID NO: 490 - protein, 49 aa, synthetic construct
  REGION 1..49: note = Modified bacterial sequence
KETLDAWAEIDHLPNLTIEQWLAFINKLDDDPSQSSELLSEAKKLNDSQ

SEQ ID NO: 491 - protein, 49 aa, synthetic construct
  REGION 1..49: note = Modified bacterial sequence
KEVIEAWDEIDKLPNLTLNQWLAFINKLDDDPSQSSELLSEAKKLNDSQ

SEQ ID NO: 492 - protein, 49 aa, synthetic construct
  REGION 1..49: note = Modified bacterial sequence
KEVLDAWNEIDQLPNLTIEQWLAFINKLDDDPSQSSELLSEAKKLNDSQ

SEQ ID NO: 493 - protein, 49 aa, synthetic construct
  REGION 1..49: note = Modified bacterial sequence
KEVLHAWNEIDHLPNLTIEQWLAFIEKLEDDPSQSSELLSEAKKLNDSQ

SEQ ID NO: 494 - protein, 49 aa, synthetic construct
  REGION 1..49: note = Modified bacterial sequence
KEVIEAWQEIDKLPNLTIDQWLAFINKLDDDPSQSSELLSEAKKLNDSQ

SEQ ID NO: 495 - protein, 49 aa, synthetic construct
  REGION 1..49: note = Modified bacterial sequence
KEVVDAWNEIDQLPNLTIEQWLAFINKLDDDPSQSSELLSEAKKLNDSQ

SEQ ID NO: 496 - protein, 49 aa, synthetic construct
  REGION 1..49: note = Modified bacterial sequence
KEQIEAWNEIDALPNLTIEQWLAFINKLADDPSQSSELLSEAKKLNDSQ

SEQ ID NO: 497 - protein, 58 aa, synthetic construct
  REGION 1..58: note = Modified bacterial sequence
VDAKYAKEVLEAWDEIDRLPNLTIEQWLAFINKLDDDPSQSSELLSEAKKLNDSQAPK

SEQ ID NO: 498 - protein, 58 aa, synthetic construct
  REGION 1..58: note = Modified bacterial sequence
VDAKYAKEVLEAWNEIDRLPNLTIEQWLAFINKLDDDPSQSSELLSEAKKLNDSQAPK

SEQ ID NO: 499 - protein, 58 aa, synthetic construct
  REGION 1..58: note = Modified bacterial sequence
VDAKYAKEVIEAWNEIDRLPNLTIEQWLAFINKLDDDPSQSSELLSEAKKLNDSQAPK

SEQ ID NO: 500 - protein, 58 aa, synthetic construct
  REGION 1..58: note = Modified bacterial sequence
VDAKYAKEVLEAWDEIDRLPNLTLDQWLAFINKLDDDPSQSSELLSEAKKLNDSQAPK

SEQ ID NO: 501 - protein, 58 aa, synthetic construct
  REGION 1..58: note = Modified bacterial sequence
VDAKYAKEVLDAWDEIDALPNLTLEQWLAFINKLDDDPSQSSELLSEAKKLNDSQAPK

SEQ ID NO: 502 - protein, 58 aa, synthetic construct
  REGION 1..58: note = Modified bacterial sequence
VDAKYAKEVIDAWDEIDRLPNLTLDQWLAFINKLDDDPSQSSELLSEAKKLNDSQAPK

SEQ ID NO: 503 - protein, 58 aa, synthetic construct
  REGION 1..58: note = Modified bacterial sequence
VDAKYAKETLEAWDEIDRLPNLTIEQWLAFINKLDDDPSQSSELLSEAKKLNDSQAPK

SEQ ID NO: 504 - protein, 58 aa, synthetic construct
  REGION 1..58: note = Modified bacterial sequence
VDAKYAKEVIDAWNEIDALPNLTLDQWLAFINKLDDDPSQSSELLSEAKKLNDSQAPK

SEQ ID NO: 505 - protein, 58 aa, synthetic construct
  REGION 1..58: note = Modified bacterial sequence
VDAKYAKEVLDAWDEIDKLPNLTIDQWLAFINKLDDDPSQSSELLSEAKKLNDSQAPK

SEQ ID NO: 506 - protein, 58 aa, synthetic construct
  REGION 1..58: note = Modified bacterial sequence
VDAKYAKEVLEAWDEIDHLPNLTLDQWLAFINKLDDDPSQSSELLSEAKKLNDSQAPK

SEQ ID NO: 507 - protein, 58 aa, synthetic construct
  REGION 1..58: note = Modified bacterial sequence
VDAKYAKEVLEAWDEIDALPNLTIEQWLAFINKLDDDPSQSSELLSEAKKLNDSQAPK

SEQ ID NO: 508 - protein, 58 aa, synthetic construct
  REGION 1..58: note = Modified bacterial sequence
VDAKYAKEVLDAWDEIDKLPNLTLEQWLAFINKLDDDPSQSSELLSEAKKLNDSQAPK

SEQ ID NO: 509 - protein, 58 aa, synthetic construct
  REGION 1..58: note = Modified bacterial sequence
VDAKYAKETITAWDEIDKLPNLTIEQWLAFIGKLEDDPSQSSELLAEAKKLNDAQAPK

SEQ ID NO: 510 - protein, 58 aa, synthetic construct
  REGION 1..58: note = Modified bacterial sequence
VDNKFNKESMKAWDEIDRLPNLNINQWVAFIDSLYDDPSQSANLLAEAKKLNDAQAPK

SEQ ID NO: 511 - protein, 58 aa, synthetic construct
  REGION 1..58: note = Modified bacterial sequence
VDAKYAKESIEAWTEIDHLPNLTIEQWLAFINKLTDDPSQSSELLAEAKKLNDAQAPK

SEQ ID NO: 512 - protein, 58 aa, synthetic construct
  REGION 1..58: note = Modified bacterial sequence
VDAKYAKEVLDAWHEIDTLPNLTVRQWLAFISKLEDDPSQSSELLAEAKKLNDAQAPK

SEQ ID NO: 513 - protein, 58 aa, synthetic construct
  REGION 1..58: note = Modified bacterial sequence
VDAKYAKEHIQANEEIDRLPNLTIKQWLAFINKLHDDPSQSSELLAEAKKLNDAQAPK

SEQ ID NO: 514 - protein, 58 aa, synthetic construct
  REGION 1..58: note = Modified bacterial sequence
VDAKYAKEVLHAWAEIDALPNLTIEQWLAFINKLDDDPSQSSELLSEAKKLNDSQAPK

SEQ ID NO: 515 - protein, 58 aa, synthetic construct
  REGION 1..58: note = Modified bacterial sequence
VDAKYAKEVLAAWDEIDSLPNLTLQQWLAFINKLDDDPSQSSELLSEAKKLNDSQAPK

SEQ ID NO: 516 - protein, 58 aa, synthetic construct
  REGION 1..58: note = Modified bacterial sequence
VDAKYAKEVIDAWNEIDALPNLTLEQWLAFINKLDDDPSQSSELLSEAKKLNDSQAPK

SEQ ID NO: 517 - protein, 58 aa, synthetic construct
  REGION 1..58: note = Modified bacterial sequence
VDAKYAKEVLDAWNEIDALPNLTIDQWLAFINKLSDDPSQSSELLSEAKKLNDSQAPK

SEQ ID NO: 518 - protein, 58 aa, synthetic construct
  REGION 1..58: note = Modified bacterial sequence
VDAKYAKEVIEAWDEIDGLPNLTIEQWLAFINKLDDDPSQSSELLSEAKKLNDSQAPK

SEQ ID NO: 519 - protein, 58 aa, synthetic construct
  REGION 1..58: note = Modified bacterial sequence
VDAKYAKEVLEAWDEIDHLPNLTLQQWLAFINKLDDDPSQSSELLSEAKKLNDSQAPK

SEQ ID NO: 520 - protein, 58 aa, synthetic construct
  REGION 1..58: note = Modified bacterial sequence
VDAKYAKEVIEAWNEIDALPNLTIEQWLAFINKLDDDPSQSSELLSEAKKLNDSQAPK

SEQ ID NO: 521 - protein, 58 aa, synthetic construct
  REGION 1..58: note = Modified bacterial sequence
VDAKYAKEVIAAWNEIDRLPNLTLTQWLAFINKLDDDPSQSSELLSEAKKLNDSQAPK

SEQ ID NO: 522 - protein, 58 aa, synthetic construct
  REGION 1..58: note = Modified bacterial sequence
VDAKYAKEVIEAWDEIDALPNLTLQQWLAFINKLDDDPSQSSELLSEAKKLNDSQAPK

SEQ ID NO: 523 - protein, 58 aa, synthetic construct
  REGION 1..58: note = Modified bacterial sequence
VDAKYAKEVIAAWDEIDKLPNLTIEQWLAFINKLDDDPSQSSELLSEAKKLNDSQAPK

SEQ ID NO: 524 - protein, 58 aa, synthetic construct
  REGION 1..58: note = Modified bacterial sequence
VDAKYAKEVIAAWDEIDKLPNLTLQQWLAFINKLDDDPSQSSELLSEAKKLNDSQAPK

SEQ ID NO: 525 - protein, 58 aa, synthetic construct
  REGION 1..58: note = Modified bacterial sequence
VDAKYAKETIAAWDEIDKLPNLTIEQWLAFINKLDDDPSQSSELLSEAKKLNDSQAPK

SEQ ID NO: 526 - protein, 58 aa, synthetic construct
  REGION 1..58: note = Modified bacterial sequence
VDAKYAKETIEAWNEIDRLPNLTIEQWLAFINKLDDDPSQSSELLSEAKKLNDSQAPK

SEQ ID NO: 527 - protein, 58 aa, synthetic construct
  REGION 1..58: note = Modified bacterial sequence
VDAKYAKEVLEAWREIDALPNLTIQQWLAFINKLDDDPSQSSELLSEAKKLNDSQAPK

SEQ ID NO: 528 - protein, 58 aa, synthetic construct
  REGION 1..58: note = Modified bacterial sequence
VDAKYAKEVIEAWDEIDQLPNLTIEQWLAFINKLDDDPSQSSELLSEAKKLNDSQAPK

SEQ ID NO: 529 - protein, 58 aa, synthetic construct
  REGION 1..58: note = Modified bacterial sequence
VDAKYAKEVLRAWDEIDHLPNLTLEQWLAFINKLDDDPSQSSELLSEAKKLNDSQAPK

SEQ ID NO: 530 - protein, 58 aa, synthetic construct
  REGION 1..58: note = Modified bacterial sequence
VDAKYAKEVLEAWDEIDRLPNLTLNQWLAFINKLDDDPSQSSELLSEAKKLNDSQAPK

SEQ ID NO: 531 - protein, 58 aa, synthetic construct
  REGION 1..58: note = Modified bacterial sequence
VDAKYAKEVLDAWNEIDHLPNLTIEQWLAFINKLDDDPSQSSELLSEAKKLNDSQAPK

SEQ ID NO: 532 - protein, 58 aa, synthetic construct
  REGION 1..58: note = Modified bacterial sequence
VDAKYAKEVIDAWNEIDKLPNLTIEQWLAFINKLDDDPSQSSELLSEAKKLNDSQAPK

SEQ ID NO: 533 - protein, 58 aa, synthetic construct
  REGION 1..58: note = Modified bacterial sequence
VDAKYAKETLEAWDEIDQLPNLTLQQWLAFINKLDDDPSQSSELLSEAKKLNDSQAPK

SEQ ID NO: 534 - protein, 58 aa, synthetic construct
  REGION 1..58: note = Modified bacterial sequence
VDAKYAKEVIEAWNEIDALPNLTLDQWLAFINKLDDDPSQSSELLSEAKKLNDSQAPK

SEQ ID NO: 535 - protein, 58 aa, synthetic construct
  REGION 1..58: note = Modified bacterial sequence
VDAKYAKEVIDAWNEIDRLPNLTLQQWLAFINKLDDDPSQSSELLSEAKKLNDSQAPK

SEQ ID NO: 536 - protein, 58 aa, synthetic construct
  REGION 1..58: note = Modified bacterial sequence
VDAKYAKEVIDAWNEIDQLPNLTLEQWLAFINKLDDDPSQSSELLSEAKKLNDSQAPK

SEQ ID NO: 537 - protein, 58 aa, synthetic construct
  REGION 1..58: note = Modified bacterial sequence
VDAKYAKETIAAWDEIDHLPNLTLEQWLAFINKLDDDPSQSSELLSEAKKLNDSQAPK

SEQ ID NO: 538 - protein, 58 aa, synthetic construct
  REGION 1..58: note = Modified bacterial sequence
VDAKYAKEVLQAWDEIDHLPNLTIQQWLAFINKLSDDPSQSSELLSEAKKLNDSQAPK

SEQ ID NO: 539 - protein, 58 aa, synthetic construct
  REGION 1..58: note = Modified bacterial sequence
VDAKYAKETLHAWAEIDRLPNLTIEQWLAFINKLDDDPSQSSELLSEAKKLNDSQAPK

SEQ ID NO: 540 - protein, 58 aa, synthetic construct
  REGION 1..58: note = Modified bacterial sequence
VDAKYAKEVLEAWNEIDHLPNLTLAQWLAFINKLDDDPSQSSELLSEAKKLNDSQAPK

SEQ ID NO: 541 - protein, 58 aa, synthetic construct
  REGION 1..58: note = Modified bacterial sequence
VDAKYAKEVIEAWDEIDKLPNLTIAQWLAFINKLDDDPSQSSELLSEAKKLNDSQAPK

SEQ ID NO: 542 - protein, 58 aa, synthetic construct
  REGION 1..58: note = Modified bacterial sequence
VDAKYAKEVLDAWDEIDHLPNLTLQQWLAFINKLDDDPSQSSELLSEAKKLNDSQAPK

SEQ ID NO: 543 - protein, 58 aa, synthetic construct
  REGION 1..58: note = Modified bacterial sequence
VDAKYAKETIEAWNEIDKLPNLTLTQWLAFINKLDDDPSQSSELLSEAKKLNDSQAPK

SEQ ID NO: 544 - protein, 58 aa, synthetic construct
  REGION 1..58: note = Modified bacterial sequence
VDAKYAKEVLEAWNEIDLLPNLTIEQWLAFINKLDDDPSQSSELLSEAKKLNDSQAPK

SEQ ID NO: 545 - protein, 58 aa, synthetic construct
  REGION 1..58: note = Modified bacterial sequence
VDAKYAKEVIEAWDEIDHLPNLTIDQWLAFINKLDDDPSQSSELLSEAKKLNDSQAPK

SEQ ID NO: 546 - protein, 58 aa, synthetic construct
  REGION 1..58: note = Modified bacterial sequence
VDAKYAKEVISAWNEIDALPNLTLQQWLAFINKLDDDPSQSSELLSEAKKLNDSQAPK

SEQ ID NO: 547 - protein, 58 aa, synthetic construct
  REGION 1..58: note = Modified bacterial sequence
VDAKYAKEVIAAWNEIDKLPNLTLEQWLAFINKLDDDPSQSSELLSEAKKLNDSQAPK

SEQ ID NO: 548 - protein, 58 aa, synthetic construct
  REGION 1..58: note = Modified bacterial sequence
VDAKYAKETIEAWNEIDSLPNLTLDQWLAFINKLDDDPSQSSELLSEAKKLNDSQAPK

SEQ ID NO: 549 - protein, 58 aa, synthetic construct
  REGION 1..58: note = Modified bacterial sequence
VDAKYAKEVLDAWNEIDQLPNLTLQQWLAFINKLDDDPSQSSELLSEAKKLNDSQAPK

SEQ ID NO: 550 - protein, 58 aa, synthetic construct
  REGION 1..58: note = Modified bacterial sequence
VDAKYAKEVLAAWNEIDHLPNLTIEQWLAFINKLDDDPSQSSELLSEAKKLNDSQAPK

SEQ ID NO: 551 - protein, 58 aa, synthetic construct
  REGION 1..58: note = Modified bacterial sequence
VDAKYAKEVLEAWDEIDHLPNLTITQWLAFINKLDDDPSQSSELLSEAKKLNDSQAPK

SEQ ID NO: 552 - protein, 58 aa, synthetic construct
  REGION 1..58: note = Modified bacterial sequence
VDAKYAKETIDAWNEIDHLPNLTIEQWLAFINKLDDDPSQSSELLSEAKKLNDSQAPK

SEQ ID NO: 553 - protein, 58 aa, synthetic construct
  REGION 1..58: note = Modified bacterial sequence
VDAKYAKEVIEAWNEIDHLPNLTIQQWLAFINKLDDDPSQSSELLSEAKKLNDSQAPK

SEQ ID NO: 554 - protein, 58 aa, synthetic construct
  REGION 1..58: note = Modified bacterial sequence
VDAKYAKEVIQAWNEIDALPNLTISQWLAFINKLDDDPSQSSELLSEAKKLNDSQAPK

SEQ ID NO: 555 - protein, 58 aa, synthetic construct
  REGION 1..58: note = Modified bacterial sequence
VDAKYAKEVIAAWDEIDSLPNLTIEQWLAFINKLDDDPSQSSELLSEAKKLNDSQAPK

SEQ ID NO: 556 - protein, 58 aa, synthetic construct
  REGION 1..58: note = Modified bacterial sequence
VDAKYAKEHIEAWNEIDALPNLTIEQWLAFINKLQDDPSQSSELLSEAKKLNDSQAPK

SEQ ID NO: 557 - protein, 58 aa, synthetic construct
  REGION 1..58: note = Modified bacterial sequence
VDAKYAKEVLEAWNEIDKLPNLTLDQWLAFINKLDDDPSQSSELLSEAKKLNDSQAPK

SEQ ID NO: 558 - protein, 58 aa, synthetic construct
  REGION 1..58: note = Modified bacterial sequence
VDAKYAKEVIDAWNEIDHLPNLTIEQWLAFINKLADDPSQSSELLSEAKKLNDSQAPK

SEQ ID NO: 559 - protein, 58 aa, synthetic construct
  REGION 1..58: note = Modified bacterial sequence
VDAKYAKETIDAWDEIDKLPNLTIEQWLAFINKLDDDPSQSSELLSEAKKLNDSQAPK

SEQ ID NO: 560 - protein, 58 aa, synthetic construct
  REGION 1..58: note = Modified bacterial sequence
VDAKYAKEVIAAWDEIDLLPNLTLQQWLAFINKLADDPSQSSELLSEAKKLNDSQAPK

SEQ ID NO: 561 - protein, 58 aa, synthetic construct
  REGION 1..58: note = Modified bacterial sequence
VDAKYAKEVIHAWDEIDKLPNLTIEQWLAFINKLDDDPSQSSELLSEAKKLNDSQAPK

SEQ ID NO: 562 - protein, 58 aa, synthetic construct
  REGION 1..58: note = Modified bacterial sequence
VDAKYAKEVIAAWNEIDHLPNLTLEQWLAFINKLDDDPSQSSELLSEAKKLNDSQAPK

SEQ ID NO: 563 - protein, 58 aa, synthetic construct
  REGION 1..58: note = Modified bacterial sequence
VDAKYAKETLDAWNEIDKLPNLTLSQWLAFINKLDDDPSQSSELLSEAKKLNDSQAPK

SEQ ID NO: 564 - protein, 58 aa, synthetic construct
  REGION 1..58: note = Modified bacterial sequence
VDAKYAKEVLEAWNEIDALPNLTLEQWLAFINKLDDDPSQSSELLSEAKKLNDSQAPK

SEQ ID NO: 565 - protein, 58 aa, synthetic construct
  REGION 1..58: note = Modified bacterial sequence
VDAKYAKEVIQAWDEIDHLPNLTISQWLAFINKLDDDPSQSSELLSEAKKLNDSQAPK

SEQ ID NO: 566 - protein, 58 aa, synthetic construct
  REGION 1..58: note = Modified bacterial sequence
VDAKYAKEVLQAWDEIDSLPNLTIEQWLAFINKLDDDPSQSSELLSEAKKLNDSQAPK

SEQ ID NO: 567 - protein, 58 aa, synthetic construct
  REGION 1..58: note = Modified bacterial sequence
VDAKYAKETLEAWDEIDHLPNLTIAQWLAFINKLDDDPSQSSELLSEAKKLNDSQAPK

SEQ ID NO: 568 - protein, 58 aa, synthetic construct
  REGION 1..58: note = Modified bacterial sequence
VDAKYAKETIDAWNEIDRLPNLTISQWLAFINKLDDDPSQSSELLSEAKKLNDSQAPK

SEQ ID NO: 569 - protein, 58 aa, synthetic construct
  REGION 1..58: note = Modified bacterial sequence
VDAKYAKEVLDAWHEIDHLPNLTIQQWLAFINKLDDDPSQSSELLSEAKKLNDSQAPK

SEQ ID NO: 570 - protein, 58 aa, synthetic construct
  REGION 1..58: note = Modified bacterial sequence
VDAKYAKEQIRAWDEIDKLPNLTIEQWLAFINKLADDPSQSSELLSEAKKLNDSQAPK

SEQ ID NO: 571 - protein, 58 aa, synthetic construct
  REGION 1..58: note = Modified bacterial sequence
VDAKYAKETLYAWNEIDKLPNLTIEQWLAFIEKLQDDPSQSSELLSEAKKLNDSQAPK

SEQ ID NO: 572 - protein, 58 aa, synthetic construct
  REGION 1..58: note = Modified bacterial sequence
VDAKYAKEVIEAWNEIDALPNLTIDQWLAFINKLDDDPSQSSELLSEAKKLNDSQAPK

SEQ ID NO: 573 - protein, 58 aa, synthetic construct
  REGION 1..58: note = Modified bacterial sequence
VDAKYAKEVLEAWNEIDHLPNLTIQQWLAFINKLDDDPSQSSELLSEAKKLNDSQAPK

SEQ ID NO: 574 - protein, 58 aa, synthetic construct
  REGION 1..58: note = Modified bacterial sequence
VDAKYAKETIEAWDEIDALPNLTIEQWLAFINKLDDDPSQSSELLSEAKKLNDSQAPK

SEQ ID NO: 575 - protein, 58 aa, synthetic construct
  REGION 1..58: note = Modified bacterial sequence
VDAKYAKEVIEAWNEIDHLPNLTLQQWLAFINKLDDDPSQSSELLSEAKKLNDSQAPK

SEQ ID NO: 576 - protein, 58 aa, synthetic construct
  REGION 1..58: note = Modified bacterial sequence
VDAKYAKEVIEAWNEIDKLPNLTIQQWLAFINKLDDDPSQSSELLSEAKKLNDSQAPK

SEQ ID NO: 577 - protein, 58 aa, synthetic construct
  REGION 1..58: note = Modified bacterial sequence
VDAKYAKETLDAWAEIDHLPNLTLDQWLAFINKLDDDPSQSSELLSEAKKLNDSQAPK

SEQ ID NO: 578 - protein, 58 aa, synthetic construct
  REGION 1..58: note = Modified bacterial sequence
VDAKYAKEHIDAWNEIDALPNLTLSQWLAFINKLDDDPSQSSELLSEAKKLNDSQAPK

SEQ ID NO: 579 - protein, 58 aa, synthetic construct
  REGION 1..58: note = Modified bacterial sequence
VDAKYAKEVLDAWNEIDKLPNLTIAQWLAFINKLDDDPSQSSELLSEAKKLNDSQAPK

SEQ ID NO: 580 - protein, 58 aa, synthetic construct
  REGION 1..58: note = Modified bacterial sequence
VDAKYAKEVIEAWTEIDYLPNLTLQQWLAFINKLDDDPSQSSELLSEAKKLNDSQAPK

SEQ ID NO: 581 - protein, 58 aa, synthetic construct
  REGION 1..58: note = Modified bacterial sequence
VDAKYAKETIEAWNEIDHLPNLTIAQWLAFINKLDDDPSQSSELLSEAKKLNDSQAPK

SEQ ID NO: 582 - protein, 58 aa, synthetic construct
  REGION 1..58: note = Modified bacterial sequence
VDAKYAKEVIQAWNEIDKLPNLTLEQWLAFINKLDDDPSQSSELLSEAKKLNDSQAPK

SEQ ID NO: 583 - protein, 58 aa, synthetic construct
  REGION 1..58: note = Modified bacterial sequence
VDAKYAKEVIEAWDEIDHLPNLTIEQWLAFINKLDDDPSQSSELLSEAKKLNDSQAPK

SEQ ID NO: 584 - protein, 58 aa, synthetic construct
  REGION 1..58: note = Modified bacterial sequence
VDAKYAKETIDAWNEIDLLPNLTIEQWLAFINKLDDDPSQSSELLSEAKKLNDSQAPK

SEQ ID NO: 585 - protein, 58 aa, synthetic construct
  REGION 1..58: note = Modified bacterial sequence
VDAKYAKEHIDAWNEIDKLPNLTLDQWLAFINKLDDDPSQSSELLSEAKKLNDSQAPK

SEQ ID NO: 586 - protein, 58 aa, synthetic construct
  REGION 1..58: note = Modified bacterial sequence
VDAKYAKEVVAAWNEIDALPNLTIEQWLAFINKLNDDPSQSSELLSEAKKLNDSQAPK

SEQ ID NO: 587 - protein, 58 aa, synthetic construct
  REGION 1..58: note = Modified bacterial sequence
VDAKYAKEVIEAWNEIDALPNLTLAQWLAFINKLDDDPSQSSELLSEAKKLNDSQAPK

SEQ ID NO: 588 - protein, 58 aa, synthetic construct
  REGION 1..58: note = Modified bacterial sequence
VDAKYAKEVLQAWDEIDRLPNLTLDQWLAFINKLDDDPSQSSELLSEAKKLNDSQAPK

SEQ ID NO: 589 - protein, 58 aa, synthetic construct
  REGION 1..58: note = Modified bacterial sequence
VDAKYAKEVIDAWDEIDHLPNLTIEQWLAFINKLSDDPSQSSELLSEAKKLNDSQAPK

SEQ ID NO: 590 - protein, 58 aa, synthetic construct
  REGION 1..58: note = Modified bacterial sequence
VDAKYAKEVVEAWNEIDQLPNLTIEQWLAFINKLDDDPSQSSELLSEAKKLNDSQAPK

SEQ ID NO: 591 - protein, 58 aa, synthetic construct
  REGION 1..58: note = Modified bacterial sequence
VDAKYAKEVIQAWNEIDALPNLTIEQWLAFINKLDDDPSQSSELLSEAKKLNDSQAPK

SEQ ID NO: 592 - protein, 58 aa, synthetic construct
  REGION 1..58: note = Modified bacterial sequence
VDAKYAKEVIQAWDEIDKLPNLTIDQWLAFINKLADDPSQSSELLSEAKKLNDSQAPK

SEQ ID NO: 593 - protein, 58 aa, synthetic construct
  REGION 1..58: note = Modified bacterial sequence
VDAKYAKEVVAAWDEIDALPNLTLTQWLAFINKLDDDPSQSSELLSEAKKLNDSQAPK

SEQ ID NO: 594 - protein, 58 aa, synthetic construct
  REGION 1..58: note = Modified bacterial sequence
VDAKYAKEVIQAWNEIDGLPNLTLSQWLAFINKLDDDPSQSSELLSEAKKLNDSQAPK

SEQ ID NO: 595 - protein, 58 aa, synthetic construct
  REGION 1..58: note = Modified bacterial sequence
VDAKYAKETIEAWDEIDALPNLTITQWLAFINKLDDDPSQSSELLSEAKKLNDSQAPK

SEQ ID NO: 596 - protein, 58 aa, synthetic construct
  REGION 1..58: note = Modified bacterial sequence
VDAKYAKEVIDAWNEIDHLPNLTIQQWLAFINKLADDPSQSSELLSEAKKLNDSQAPK

SEQ ID NO: 597 - protein, 58 aa, synthetic construct
  REGION 1..58: note = Modified bacterial sequence
VDAKYAKETIEAWNEIDALPNLTLDQWLAFINKLEDDPSQSSELLSEAKKLNDSQAPK

SEQ ID NO: 598 - protein, 58 aa, synthetic construct
  REGION 1..58: note = Modified bacterial sequence
VDAKYAKEHIHAWNEIDELPNLTIEQWLAFINKLADDPSQSSELLSEAKKLNDSQAPK

SEQ ID NO: 599 - protein, 58 aa, synthetic construct
  REGION 1..58: note = Modified bacterial sequence
VDAKYAKEVIDAWDEIDHLPNLTIDQWLAFINKLSDDPSQSSELLSEAKKLNDSQAPK

SEQ ID NO: 600 - protein, 58 aa, synthetic construct
  REGION 1..58: note = Modified bacterial sequence
VDAKYAKEVIDANDEIDALPNLTIAQWLAFINKLHDDPSQSSELLSEAKKLNDSQAPK

SEQ ID NO: 601 - protein, 58 aa, synthetic construct
  REGION 1..58: note = Modified bacterial sequence
VDAKYAKETIEAWDEIDKLPNLTIEQWLAFINKLDDDPSQSSELLSEAKKLNDSQAPK

SEQ ID NO: 602 - protein, 58 aa, synthetic construct
  REGION 1..58: note = Modified bacterial sequence
VDAKYAKEVLLAWDEIDHLPNLTLEQWLAFINKLDDDPSQSSELLSEAKKLNDSQAPK

SEQ ID NO: 603 - protein, 58 aa, synthetic construct
  REGION 1..58: note = Modified bacterial sequence
VDAKYAKEHIDAWNEIDGLPNLTLEQWLAFINKLDDDPSQSSELLSEAKKLNDSQAPK

SEQ ID NO: 604 - protein, 58 aa, synthetic construct
  REGION 1..58: note = Modified bacterial sequence
VDAKYAKEVIEAWSEIDALPNLTIDQWLAFINKLADDPSQSSELLSEAKKLNDSQAPK

SEQ ID NO: 605 - protein, 58 aa, synthetic construct
  REGION 1..58: note = Modified bacterial sequence
VDAKYAKEQLNAWAEIDALPNLTIEQWLAFINKLDDDPSQSSELLSEAKKLNDSQAPK

SEQ ID NO: 606 - protein, 58 aa, synthetic construct
  REGION 1..58: note = Modified bacterial sequence
VDAKYAKEVIDAWNEIDALPNLTIAQWLAFINKLDDDPSQSSELLSEAKKLNDSQAPK

SEQ ID NO: 607 - protein, 58 aa, synthetic construct
  REGION 1..58: note = Modified bacterial sequence
VDAKYAKETIDAWNEIDQLPNLTIEQWLAFINKLDDDPSQSSELLSEAKKLNDSQAPK

SEQ ID NO: 608 - protein, 58 aa, synthetic construct
  REGION 1..58: note = Modified bacterial sequence
VDAKYAKEVIEAWDEIDKLPNLTLAQWLAFINKLDDDPSQSSELLSEAKKLNDSQAPK

SEQ ID NO: 609 - protein, 58 aa, synthetic construct
  REGION 1..58: note = Modified bacterial sequence
VDAKYAKEVLYAWAEIDHLPNLTIEQWLAFINKLDDDPSQSSELLSEAKKLNDSQAPK

SEQ ID NO: 610 - protein, 58 aa, synthetic construct
  REGION 1..58: note = Modified bacterial sequence
VDAKYAKEQIDAWNEIDRLPNLTIQQWLAFINKLDDDPSQSSELLSEAKKLNDSQAPK

SEQ ID NO: 611 - protein, 58 aa, synthetic construct
  REGION 1..58: note = Modified bacterial sequence
VDAKYAKEVLAAWDEIDRLPNLTIEQWLAFINKLDDDPSQSSELLSEAKKLNDSQAPK

SEQ ID NO: 612 - protein, 58 aa, synthetic construct
  REGION 1..58: note = Modified bacterial sequence
VDAKYAKEVIEAWDEIDHLPNLTLHQWLAFINKLDDDPSQSSELLSEAKKLNDSQAPK

SEQ ID NO: 613 - protein, 58 aa, synthetic construct
  REGION 1..58: note = Modified bacterial sequence
VDAKYAKEVIEAWNEIDKLPNLTLQQWLAFINKLDDDPSQSSELLSEAKKLNDSQAPK

SEQ ID NO: 614 - protein, 58 aa, synthetic construct
  REGION 1..58: note = Modified bacterial sequence
VDAKYAKEVIDANDEIDALPNLTIEQWLAFINKLHDDPSQSSELLSEAKKLNDSQAPK

SEQ ID NO: 615 - protein, 58 aa, synthetic construct
  REGION 1..58: note = Modified bacterial sequence
VDAKYAKEVIAAWDEIDALPNLTIEQWLAFINKLDDDPSQSSELLSEAKKLNDSQAPK

SEQ ID NO: 616 - protein, 58 aa, synthetic construct
  REGION 1..58: note = Modified bacterial sequence
VDAKYAKEVIEAWTEIDQLPNLTLDQWLAFINKLDDDPSQSSELLSEAKKLNDSQAPK

SEQ ID NO: 617 - protein, 58 aa, synthetic construct
  REGION 1..58: note = Modified bacterial sequence
VDAKYAKEVINAWNEIDALPNLTLQQWLAFINKLDDDPSQSSELLSEAKKLNDSQAPK

SEQ ID NO: 618 - protein, 58 aa, synthetic construct
  REGION 1..58: note = Modified bacterial sequence
VDAKYAKEHIEAWDEIDHLPNLTIDQWLAFINKLADDPSQSSELLSEAKKLNDSQAPK

SEQ ID NO: 619 - protein, 58 aa, synthetic construct
  REGION 1..58: note = Modified bacterial sequence
VDAKYAKEHLEAWREIDALPNLTIEQWLAFINKLDDDPSQSSELLSEAKKLNDSQAPK

SEQ ID NO: 620 - protein, 58 aa, synthetic construct
  REGION 1..58: note = Modified bacterial sequence
VDAKYAKEVLDAWNEIDKLPNLTLQQWLAFINKLDDDPSQSSELLSEAKKLNDSQAPK

SEQ ID NO: 621 - protein, 58 aa, synthetic construct
  REGION 1..58: note = Modified bacterial sequence
VDAKYAKEVIAAWDEIDHLPNLTIQQWLAFINKLDDDPSQSSELLSEAKKLNDSQAPK

SEQ ID NO: 622 - protein, 58 aa, synthetic construct
  REGION 1..58: note = Modified bacterial sequence
VDAKYAKEVIQAWNEIDALPNLTLEQWLAFINKLDDDPSQSSELLSEAKKLNDSQAPK

SEQ ID NO: 623 - protein, 58 aa, synthetic construct
  REGION 1..58: note = Modified bacterial sequence
VDAKYAKEVIDAWNEIDHLPNLTIAQWLAFINKLDDDPSQSSELLSEAKKLNDSQAPK

SEQ ID NO: 624 - protein, 58 aa, synthetic construct
  REGION 1..58: note = Modified bacterial sequence
VDAKYAKEQLDAWDEIDHLPNLTIDQWLAFINKLSDDPSQSSELLSEAKKLNDSQAPK

SEQ ID NO: 625 - protein, 58 aa, synthetic construct
  REGION 1..58: note = Modified bacterial sequence
VDAKYAKEVLNAWDEIDKLPNLTIEQWLAFINKLDDDPSQSSELLSEAKKLNDSQAPK

SEQ ID NO: 626 - protein, 58 aa, synthetic construct
  REGION 1..58: note = Modified bacterial sequence
VDAKYAKEVLEAWNEIDHLPNLTIDQWLAFINKLDDDPSQSSELLSEAKKLNDSQAPK

SEQ ID NO: 627 - protein, 58 aa, synthetic construct
  REGION 1..58: note = Modified bacterial sequence
VDAKYAKEVLLAWDEIDRLPNLTIDQWLAFINKLADDPSQSSELLSEAKKLNDSQAPK

SEQ ID NO: 628 - protein, 58 aa, synthetic construct
  REGION 1..58: note = Modified bacterial sequence
VDAKYAKEVIAAWNEIDQLPNLTLDQWLAFINKLDDDPSQSSELLSEAKKLNDSQAPK

SEQ ID NO: 629 - protein, 58 aa, synthetic construct
  REGION 1..58: note = Modified bacterial sequence
VDAKYAKETLLAWDEIDALPNLTIEQWLAFINKLDDDPSQSSELLSEAKKLNDSQAPK

SEQ ID NO: 630 - protein, 58 aa, synthetic construct
  REGION 1..58: note = Modified bacterial sequence
VDAKYAKEVIDAWNEIDTLPNLTLEQWLAFINKLDDDPSQSSELLSEAKKLNDSQAPK

SEQ ID NO: 631 - protein, 58 aa, synthetic construct
  REGION 1..58: note = Modified bacterial sequence
VDAKYAKEVLHAWNEIDHLPNLTLNQWLAFINKLQDDPSQSSELLSEAKKLNDSQAPK

SEQ ID NO: 632 - protein, 58 aa, synthetic construct
  REGION 1..58: note = Modified bacterial sequence
VDAKYAKEVIQAWNEIDALPNLTIAQWLAFINKLDDDPSQSSELLSEAKKLNDSQAPK

SEQ ID NO: 633 - protein, 58 aa, synthetic construct
  REGION 1..58: note = Modified bacterial sequence
VDAKYAKETVDAWNEIDALPNLTIEQWLAFINKLDDDPSQSSELLSEAKKLNDSQAPK

SEQ ID NO: 634 - protein, 58 aa, synthetic construct
  REGION 1..58: note = Modified bacterial sequence
VDAKYAKEVIQAWDEIDHLPNLTIDQWLAFINKLDDDPSQSSELLSEAKKLNDSQAPK

SEQ ID NO: 635 - protein, 58 aa, synthetic construct
  REGION 1..58: note = Modified bacterial sequence
VDAKYAKEVLDAWNEIDQLPNLTIQQWLAFINKLDDDPSQSSELLSEAKKLNDSQAPK

SEQ ID NO: 636 - protein, 58 aa, synthetic construct
  REGION 1..58: note = Modified bacterial sequence
VDAKYAKETIEAWNEIDALPNLTLDQWLAFINKLDDDPSQSSELLSEAKKLNDSQAPK

SEQ ID NO: 637 - protein, 58 aa, synthetic construct
  REGION 1..58: note = Modified bacterial sequence
VDAKYAKEVIEAWDEIDALPNLTIDQWLAFINKLDDDPSQSSELLSEAKKLNDSQAPK

SEQ ID NO: 638 - protein, 58 aa, synthetic construct
  REGION 1..58: note = Modified bacterial sequence
VDAKYAKEVIEAWNEIDQLPNLTIQQWLAFINKLDDDPSQSSELLSEAKKLNDSQAPK

SEQ ID NO: 639 - protein, 58 aa, synthetic construct
  REGION 1..58: note = Modified bacterial sequence
VDAKYAKEVIEAWTEIDHLPNLTIEQWLAFINKLDDDPSQSSELLSEAKKLNDSQAPK

SEQ ID NO: 640 - protein, 58 aa, synthetic construct
  REGION 1..58: note = Modified bacterial sequence
VDAKYAKEVIQAWNEIDHLPNLTLQQWLAFINKLEDDPSQSSELLSEAKKLNDSQAPK

SEQ ID NO: 641 - protein, 58 aa, synthetic construct
  REGION 1..58: note = Modified bacterial sequence
VDAKYAKEVIQANNEIDQLPNLTIEQWLAFINKLHDDPSQSSELLSEAKKLNDSQAPK

SEQ ID NO: 642 - protein, 58 aa, synthetic construct
  REGION 1..58: note = Modified bacterial sequence
VDAKYAKEVLHAWSEIDKLPNLTIEQWLAFINKLDDDPSQSSELLSEAKKLNDSQAPK

SEQ ID NO: 643 - protein, 58 aa, synthetic construct
  REGION 1..58: note = Modified bacterial sequence
VDAKYAKETIQAWDEIDKLPNLTLDQWLAFINKLSDDPSQSSELLSEAKKLNDSQAPK

SEQ ID NO: 644 - protein, 58 aa, synthetic construct
  REGION 1..58: note = Modified bacterial sequence
VDAKYAKETLRAWDEIDKLPNLTIQQWLAFINKLADDPSQSSELLSEAKKLNDSQAPK

SEQ ID NO: 645 - protein, 58 aa, synthetic construct
  REGION 1..58: note = Modified bacterial sequence
VDAKYAKEVIDAWNEIDHLPNLTIEQWLAFINKLEDDPSQSSELLSEAKKLNDSQAPK

SEQ ID NO: 646 - protein, 58 aa, synthetic construct
  REGION 1..58: note = Modified bacterial sequence
VDAKYAKEVIDAWNEIDHLPNLTLQQWLAFINKLADDPSQSSELLSEAKKLNDSQAPK

SEQ ID NO: 647 - protein, 58 aa, synthetic construct
  REGION 1..58: note = Modified bacterial sequence
VDAKYAKETIDAWNEIDALPNLTLDQWLAFINKLDDDPSQSSELLSEAKKLNDSQAPK

SEQ ID NO: 648 - protein, 58 aa, synthetic construct
  REGION 1..58: note = Modified bacterial sequence
VDAKYAKEVIEAWNEIDQLPNLTIEQWLAFINKLDDDPSQSSELLSEAKKLNDSQAPK

SEQ ID NO: 649 - protein, 58 aa, synthetic construct
  REGION 1..58: note = Modified bacterial sequence
VDAKYAKEVIRAWDEIDQLPNLTLSQWLAFINKLDDDPSQSSELLSEAKKLNDSQAPK

SEQ ID NO: 650 - protein, 58 aa, synthetic construct
  REGION 1..58: note = Modified bacterial sequence
VDAKYAKEVIEAWNEIDRLPNLTIHQWLAFINKLDDDPSQSSELLSEAKKLNDSQAPK

SEQ ID NO: 651 - protein, 58 aa, synthetic construct
  REGION 1..58: note = Modified bacterial sequence
VDAKYAKETIEAWNEIDQLPNLTIEQWLAFINKLDDDPSQSSELLSEAKKLNDSQAPK

SEQ ID NO: 652 - protein, 58 aa, synthetic construct
  REGION 1..58: note = Modified bacterial sequence
VDAKYAKEVLTAWAEIDALPNLTLSQWLAFINKLDDDPSQSSELLSEAKKLNDSQAPK

SEQ ID NO: 653 - protein, 58 aa, synthetic construct
  REGION 1..58: note = Modified bacterial sequence
VDAKYAKEVIEAWDEIDKLPNLTVDQWLAFINKLDDDPSQSSELLSEAKKLNDSQAPK

SEQ ID NO: 654 - protein, 58 aa, synthetic construct
  REGION 1..58: note = Modified bacterial sequence
VDAKYAKEVIDAWNEIDHLPNLTLTQWLAFINKLDDDPSQSSELLSEAKKLNDSQAPK

SEQ ID NO: 655 - protein, 58 aa, synthetic construct
  REGION 1..58: note = Modified bacterial sequence
VDAKYAKEVIEAWNEIDQLPNLTLDQWLAFINKLDDDPSQSSELLSEAKKLNDSQAPK

SEQ ID NO: 656 - protein, 58 aa, synthetic construct
  REGION 1..58: note = Modified bacterial sequence
VDAKYAKETLQAWDEIDHLPNLTLNQWLAFINKLDDDPSQSSELLSEAKKLNDSQAPK

SEQ ID NO: 657 - protein, 58 aa, synthetic construct
  REGION 1..58: note = Modified bacterial sequence
VDAKYAKEVIDAWNEIDHLPNLTIEQWLAFINKLDDDPSQSSELLSEAKKLNDSQAPK

SEQ ID NO: 658 - protein, 58 aa, synthetic construct
  REGION 1..58: note = Modified bacterial sequence
VDAKYAKEVIEAWNEIDLLPNLTLSQWLAFINKLDDDPSQSSELLSEAKKLNDSQAPK

SEQ ID NO: 659 - protein, 58 aa, synthetic construct
  REGION 1..58: note = Modified bacterial sequence
VDAKYAKEVIDAWDEIDRLPNLTLKQWLAFINKLDDDPSQSSELLSEAKKLNDSQAPK

SEQ ID NO: 660 - protein, 58 aa, synthetic construct
  REGION 1..58: note = Modified bacterial sequence
VDAKYAKETLHAWDEIDKLPNLTIEQWLAFINKLDDDPSQSSELLSEAKKLNDSQAPK

SEQ ID NO: 661 - protein, 58 aa, synthetic construct
  REGION 1..58: note = Modified bacterial sequence
VDAKYAKEVIKAWDEIDHLPNLTLNQWLAFINKLDDDPSQSSELLSEAKKLNDSQAPK

SEQ ID NO: 662 - protein, 58 aa, synthetic construct
  REGION 1..58: note = Modified bacterial sequence
VDAKYAKEVIEAWNEIDHLPNLTLAQWLAFINKLDDDPSQSSELLSEAKKLNDSQAPK

SEQ ID NO: 663 - protein, 58 aa, synthetic construct
  REGION 1..58: note = Modified bacterial sequence
VDAKYAKEVIQAWNEIDHLPNLTIDQWLAFITKLEDDPSQSSELLSEAKKLNDSQAPK

SEQ ID NO: 664 - protein, 58 aa, synthetic construct
  REGION 1..58: note = Modified bacterial sequence
VDAKYAKEVIEAWNEIDRLPNLTIKQWLAFINKLDDDPSQSSELLSEAKKLNDSQAPK

SEQ ID NO: 665 - protein, 58 aa, synthetic construct
  REGION 1..58: note = Modified bacterial sequence
VDAKYAKEVIEAWNEIDSLPNLTLQQWLAFINKLDDDPSQSSELLSEAKKLNDSQAPK

SEQ ID NO: 666 - protein, 58 aa, synthetic construct
  REGION 1..58: note = Modified bacterial sequence
VDAKYAKETIDAWNEIDKLPNLTIEQWLAFINKLDDDPSQSSELLSEAKKLNDSQAPK

SEQ ID NO: 667 - protein, 58 aa, synthetic construct
  REGION 1..58: note = Modified bacterial sequence
VDAKYAKEVLEAWAEIDALPNLTIAQWLAFINKLDDDPSQSSELLSEAKKLNDSQAPK

SEQ ID NO: 668 - protein, 58 aa, synthetic construct
  REGION 1..58: note = Modified bacterial sequence
VDAKYAKETIDAWNEIDRLPNLTIEQWLAFINKLDDDPSQSSELLSEAKKLNDSQAPK

SEQ ID NO: 669 - protein, 58 aa, synthetic construct
  REGION 1..58: note = Modified bacterial sequence
VDAKYAKETLKAWDEIDRLPNLTLEQWLAFINKLDDDPSQSSELLSEAKKLNDSQAPK

SEQ ID NO: 670 - protein, 58 aa, synthetic construct
  REGION 1..58: note = Modified bacterial sequence
VDAKYAKETIAAWNEIDALPNLTLQQWLAFINKLDDDPSQSSELLSEAKKLNDSQAPK

SEQ ID NO: 671 - protein, 58 aa, synthetic construct
  REGION 1..58: note = Modified bacterial sequence
VDAKYAKEVLQAWNEIDHLPNLTIQQWLAFINKLDDDPSQSSELLSEAKKLNDSQAPK

SEQ ID NO: 672 - protein, 58 aa, synthetic construct
  REGION 1..58: note = Modified bacterial sequence
VDAKYAKEVIEAWSEIDHLPNLTLQQWLAFINKLDDDPSQSSELLSEAKKLNDSQAPK

SEQ ID NO: 673 - protein, 58 aa, synthetic construct
  REGION 1..58: note = Modified bacterial sequence
VDAKYAKEVIDAWNEIDGLPNLTIEQWLAFINKLDDDPSQSSELLSEAKKLNDSQAPK

SEQ ID NO: 674 - protein, 58 aa, synthetic construct
  REGION 1..58: note = Modified bacterial sequence
VDAKYAKEVIHAWNEIDHLPNLTLNQWLAFINKLEDDPSQSSELLSEAKKLNDSQAPK

SEQ ID NO: 675 - protein, 58 aa, synthetic construct
  REGION 1..58: note = Modified bacterial sequence
VDAKYAKEVLDAWNEIDSLPNLTLDQWLAFINKLDDDPSQSSELLSEAKKLNDSQAPK

SEQ ID NO: 676 - protein, 58 aa, synthetic construct
  REGION 1..58: note = Modified bacterial sequence
VDAKYAKEQIEAWNEIDRLPNLTLEQWLAFINKLDDDPSQSSELLSEAKKLNDSQAPK

SEQ ID NO: 677 - protein, 58 aa, synthetic construct
  REGION 1..58: note = Modified bacterial sequence
VDAKYAKEVVDAWNEIDALPNLTLQQWLAFINKLDDDPSQSSELLSEAKKLNDSQAPK

SEQ ID NO: 678 - protein, 58 aa, synthetic construct
  REGION 1..58: note = Modified bacterial sequence
VDAKYAKEVIEAWNEIDKLPNLTIEQWLAFINKLDDDPSQSSELLSEAKKLNDSQAPK

SEQ ID NO: 679 - protein, 58 aa, synthetic construct
  REGION 1..58: note = Modified bacterial sequence
VDAKYAKEVIEANDEIDRLPNLTIEQWLAFINKLHDDPSQSSELLSEAKKLNDSQAPK

SEQ ID NO: 680 - protein, 58 aa, synthetic construct
  REGION 1..58: note = Modified bacterial sequence
VDAKYAKETLQAWDEIDKLPNLTIEQWLAFINKLDDDPSQSSELLSEAKKLNDSQAPK

SEQ ID NO: 681 - protein, 58 aa, synthetic construct
  REGION 1..58: note = Modified bacterial sequence
VDAKYAKEVIEAWDEIDHLPNLTIDQWLAFINKLADDPSQSSELLSEAKKLNDSQAPK

SEQ ID NO: 682 - protein, 58 aa, synthetic construct
  REGION 1..58: note = Modified bacterial sequence
VDAKYAKETIDAWNEIDHLPNLTLQQWLAFINKLADDPSQSSELLSEAKKLNDSQAPK

SEQ ID NO: 683 - protein, 58 aa, synthetic construct
  REGION 1..58: note = Modified bacterial sequence
VDAKYAKEVIDAWDEIDKLPNLTIEQWLAFINKLDDDPSQSSELLSEAKKLNDSQAPK

SEQ ID NO: 684 - protein, 58 aa, synthetic construct
  REGION 1..58: note = Modified bacterial sequence
VDAKYAKEVIEAWNEIDKLPNLTLAQWLAFINKLDDDPSQSSELLSEAKKLNDSQAPK

SEQ ID NO: 685 - protein, 58 aa, synthetic construct
  REGION 1..58: note = Modified bacterial sequence
VDAKYAKEVLQAWDEIDKLPNLTIQQWLAFINKLDDDPSQSSELLSEAKKLNDSQAPK

SEQ ID NO: 686 - protein, 58 aa, synthetic construct
  REGION 1..58: note = Modified bacterial sequence
VDAKYAKEVIAAWNEIDGLPNLTLQQWLAFINKLDDDPSQSSELLSEAKKLNDSQAPK

SEQ ID NO: 687 - protein, 58 aa, synthetic construct
  REGION 1..58: note = Modified bacterial sequence
VDAKYAKETLNAWNEIDALPNLTLQQWLAFINKLDDDPSQSSELLSEAKKLNDSQAPK

SEQ ID NO: 688 - protein, 58 aa, synthetic construct
  REGION 1..58: note = Modified bacterial sequence
VDAKYAKEVLSAWNEIDQLPNLTLEQWLAFINKLDDDPSQSSELLSEAKKLNDSQAPK

SEQ ID NO: 689 - protein, 58 aa, synthetic construct
  REGION 1..58: note = Modified bacterial sequence
VDAKYAKETLEAWDEIDHLPNLTLHQWLAFINKLDDDPSQSSELLSEAKKLNDSQAPK

SEQ ID NO: 690 - protein, 58 aa, synthetic construct
  REGION 1..58: note = Modified bacterial sequence
VDAKYAKEQIEAWNEIDHLPNLTLQQWLAFINKLADDPSQSSELLSEAKKLNDSQAPK

SEQ ID NO: 691 - protein, 58 aa, synthetic construct
  REGION 1..58: note = Modified bacterial sequence
VDAKYAKEVVEAWDEIDKLPNLTIEQWLAFINKLDDDPSQSSELLSEAKKLNDSQAPK

SEQ ID NO: 692 - protein, 58 aa, synthetic construct
  REGION 1..58: note = Modified bacterial sequence
VDAKYAKEVLEAWNEIDELPNLTIEQWLAFINKLDDDPSQSSELLSEAKKLNDSQAPK

SEQ ID NO: 693 - protein, 58 aa, synthetic construct
  REGION 1..58: note = Modified bacterial sequence
VDAKYAKEVIDAWNEIDQLPNLTLQQWLAFINKLDDDPSQSSELLSEAKKLNDSQAPK

SEQ ID NO: 694 - protein, 58 aa, synthetic construct
  REGION 1..58: note = Modified bacterial sequence
VDAKYAKETIDAWDEIDKLPNLTLSQWLAFINKLDDDPSQSSELLSEAKKLNDSQAPK

SEQ ID NO: 695 - protein, 58 aa, synthetic construct
  REGION 1..58: note = Modified bacterial sequence
VDAKYAKETIDAWNEIDQLPNLTLQQWLAFINKLDDDPSQSSELLSEAKKLNDSQAPK

SEQ ID NO: 696 - protein, 58 aa, synthetic construct
  REGION 1..58: note = Modified bacterial sequence
VDAKYAKEVIQAWDEIDALPNLTLNQWLAFINKLDDDPSQSSELLSEAKKLNDSQAPK

SEQ ID NO: 697 - protein, 58 aa, synthetic construct
  REGION 1..58: note = Modified bacterial sequence
VDAKYAKEVLDAWAEIDQLPNLTLQQWLAFINKLDDDPSQSSELLSEAKKLNDSQAPK

SEQ ID NO: 698 - protein, 58 aa, synthetic construct
  REGION 1..58: note = Modified bacterial sequence
VDAKYAKEHIAAWDEIDALPNLTIEQWLAFINKLDDDPSQSSELLSEAKKLNDSQAPK

SEQ ID NO: 699 - protein, 58 aa, synthetic construct
  REGION 1..58: note = Modified bacterial sequence
VDAKYAKEVIRAWDEIDALPNLTIEQWLAFINKLDDDPSQSSELLSEAKKLNDSQAPK

SEQ ID NO: 700 - protein, 58 aa, synthetic construct
  REGION 1..58: note = Modified bacterial sequence
VDAKYAKEVIDAWDEIDALPNLTIDQWLAFINKLADDPSQSSELLSEAKKLNDSQAPK

SEQ ID NO: 701 - protein, 58 aa, synthetic construct
  REGION 1..58: note = Modified bacterial sequence
VDAKYAKEVIDAWNEIDRLPNLTIQQWLAFINKLDDDPSQSSELLSEAKKLNDSQAPK

SEQ ID NO: 702 - protein, 58 aa, synthetic construct
  REGION 1..58: note = Modified bacterial sequence
VDAKYAKEVITAWNEIDHLPNLTLSQWLAFINKLDDDPSQSSELLSEAKKLNDSQAPK

SEQ ID NO: 703 - protein, 58 aa, synthetic construct
  REGION 1..58: note = Modified bacterial sequence
VDAKYAKEVIDAWNEIDALPNLTIHQWLAFINKLDDDPSQSSELLSEAKKLNDSQAPK

SEQ ID NO: 704 - protein, 58 aa, synthetic construct
  REGION 1..58: note = Modified bacterial sequence
VDAKYAKEQLKAWDEIDKLPNLTIEQWLAFIEKLQDDPSQSSELLSEAKKLNDSQAPK

SEQ ID NO: 705 - protein, 58 aa, synthetic construct
  REGION 1..58: note = Modified bacterial sequence
VDAKYAKEHIDAWTEIDHLPNLTIEQWLAFINKLDDDPSQSSELLSEAKKLNDSQAPK

SEQ ID NO: 706 - protein, 58 aa, synthetic construct
  REGION 1..58: note = Modified bacterial sequence
VDAKYAKEQLRAWDEIDKLPNLTIEQWLAFINKLQDDPSQSSELLSEAKKLNDSQAPK

SEQ ID NO: 707 - protein, 58 aa, synthetic construct
  REGION 1..58: note = Modified bacterial sequence
VDAKYAKEVLEAWREIDSLPNLTIAQWLAFINKLDDDPSQSSELLSEAKKLNDSQAPK

SEQ ID NO: 708 - protein, 58 aa, synthetic construct
  REGION 1..58: note = Modified bacterial sequence
VDAKYAKEVIQAWNEIDKLPNLTIEQWLAFINKLDDDPSQSSELLSEAKKLNDSQAPK

SEQ ID NO: 709 - protein, 58 aa, synthetic construct
  REGION 1..58: note = Modified bacterial sequence
VDAKYAKEHVEAWNEIDQLPNLTIEQWLAFINKLADDPSQSSELLSEAKKLNDSQAPK

SEQ ID NO: 710 - protein, 58 aa, synthetic construct
  REGION 1..58: note = Modified bacterial sequence
VDAKYAKEVIDAWDEIDALPNLTIDQWLAFINKLSDDPSQSSELLSEAKKLNDSQAPK

SEQ ID NO: 711 - protein, 58 aa, synthetic construct
  REGION 1..58: note = Modified bacterial sequence
VDAKYAKEVIEAWNEIDHLPNLTIEQWLAFINKLDDDPSQSSELLSEAKKLNDSQAPK

SEQ ID NO: 712 - protein, 58 aa, synthetic construct
  REGION 1..58: note = Modified bacterial sequence
VDAKYAKEVLQAWDEIDKLPNLTIEQWLAFINKLSDDPSQSSELLSEAKKLNDSQAPK

SEQ ID NO: 713 - protein, 58 aa, synthetic construct
  REGION 1..58: note = Modified bacterial sequence
VDAKYAKEVIKAWNEIDSLPNLTIEQWLAFINKLDDDPSQSSELLSEAKKLNDSQAPK

SEQ ID NO: 714 - protein, 58 aa, synthetic construct
  REGION 1..58: note = Modified bacterial sequence
VDAKYAKEVLEAWHEIDLLPNLTIQQWLAFINKLDDDPSQSSELLSEAKKLNDSQAPK

SEQ ID NO: 715 - protein, 58 aa, synthetic construct
  REGION 1..58: note = Modified bacterial sequence
VDAKYAKEVLEAWTEIDRLPNLTLDQWLAFINKLDDDPSQSSELLSEAKKLNDSQAPK

SEQ ID NO: 716 - protein, 58 aa, synthetic construct
  REGION 1..58: note = Modified bacterial sequence
VDAKYAKEQLYAWNEIDHLPNLTIEQWLAFIEKLQDDPSQSSELLSEAKKLNDSQAPK

SEQ ID NO: 717 - protein, 58 aa, synthetic construct
  REGION 1..58: note = Modified bacterial sequence
VDAKYAKEVLNAWDEIDKLPNLTIKQWLAFINKLDDDPSQSSELLSEAKKLNDSQAPK

SEQ ID NO: 718 - protein, 58 aa, synthetic construct
  REGION 1..58: note = Modified bacterial sequence
VDAKYAKEVIRAWDEIDKLPNLTVEQWLAFINKLDDDPSQSSELLSEAKKLNDSQAPK

SEQ ID NO: 719 - protein, 58 aa, synthetic construct
  REGION 1..58: note = Modified bacterial sequence
VDAKYAKEVVQAWDEIDQLPNLTLEQWLAFINKLDDDPSQSSELLSEAKKLNDSQAPK

SEQ ID NO: 720 - protein, 58 aa, synthetic construct
  REGION 1..58: note = Modified bacterial sequence
VDAKYAKEVIRAWDEIDQLPNLTLEQWLAFINKLDDDPSQSSELLSEAKKLNDSQAPK

SEQ ID NO: 721 - protein, 58 aa, synthetic construct
  REGION 1..58: note = Modified bacterial sequence
VDAKYAKETIDAWNEIDHLPNLTLDQWLAFINKLDDDPSQSSELLSEAKKLNDSQAPK

SEQ ID NO: 722 - protein, 58 aa, synthetic construct
  REGION 1..58: note = Modified bacterial sequence
VDAKYAKEVVAAWTEIDLLPNLTLDQWLAFINKLEDDPSQSSELLSEAKKLNDSQAPK

SEQ ID NO: 723 - protein, 58 aa, synthetic construct
  REGION 1..58: note = Modified bacterial sequence
VDAKYAKEVVAAWDEIDALPNLTIEQWLAFINKLSDDPSQSSELLSEAKKLNDSQAPK

SEQ ID NO: 724 - protein, 58 aa, synthetic construct
  REGION 1..58: note = Modified bacterial sequence
VDAKYAKETLEAWREIDSLPNLTLEQWLAFINKLDDDPSQSSELLSEAKKLNDSQAPK

SEQ ID NO: 725 - protein, 58 aa, synthetic construct
  REGION 1..58: note = Modified bacterial sequence
VDAKYAKEVIKAWNEIDHLPNLTLDQWLAFINKLDDDPSQSSELLSEAKKLNDSQAPK

SEQ ID NO: 726 - protein, 58 aa, synthetic construct
  REGION 1..58: note = Modified bacterial sequence
VDAKYAKEVLEAWTEIDKLPNLTIDQWLAFINKLDDDPSQSSELLSEAKKLNDSQAPK

SEQ ID NO: 727 - protein, 58 aa, synthetic construct
  REGION 1..58: note = Modified bacterial sequence
VDAKYAKETLEAWDEIDKLPNLTIDQWLAFINKLDDDPSQSSELLSEAKKLNDSQAPK

SEQ ID NO: 728 - protein, 58 aa, synthetic construct
  REGION 1..58: note = Modified bacterial sequence
VDAKYAKEVIEAWNEIDKLPNLTIDQWLAFINKLDDDPSQSSELLSEAKKLNDSQAPK

SEQ ID NO: 729 - protein, 58 aa, synthetic construct
  REGION 1..58: note = Modified bacterial sequence
VDAKYAKETIDAWNEIDKLPNLTLEQWLAFINKLDDDPSQSSELLSEAKKLNDSQAPK

SEQ ID NO: 730 - protein, 58 aa, synthetic construct
  REGION 1..58: note = Modified bacterial sequence
VDAKYAKETLDAWDEIDALPNLTIDQWLAFINKLEDDPSQSSELLSEAKKLNDSQAPK

SEQ ID NO: 731 - protein, 58 aa, synthetic construct
  REGION 1..58: note = Modified bacterial sequence
VDAKYAKEVLSAWNEIDHLPNLTIQQWLAFINKLDDDPSQSSELLSEAKKLNDSQAPK

SEQ ID NO: 732 - protein, 58 aa, synthetic construct
  REGION 1..58: note = Modified bacterial sequence
VDAKYAKEVIQANDEIDKLPNLTIEQWLAFIHKLHDDPSQSSELLSEAKKLNDSQAPK

SEQ ID NO: 733 - protein, 58 aa, synthetic construct
  REGION 1..58: note = Modified bacterial sequence
VDAKYAKEHLDAWDEIDHLPNLTIQQWLAFINKLADDPSQSSELLSEAKKLNDSQAPK

SEQ ID NO: 734 - protein, 58 aa, synthetic construct
  REGION 1..58: note = Modified bacterial sequence
VDAKYAKEVIQAWNEIDQLPNLTIEQWLAFINKLDDDPSQSSELLSEAKKLNDSQAPK

SEQ ID NO: 735 - protein, 58 aa, synthetic construct
  REGION 1..58: note = Modified bacterial sequence
VDAKYAKEVIEAWNEIDYLPNLTIAQWIAFINKLDDDPSQSSELLSEAKKLNDSQAPK

SEQ ID NO: 736 - protein, 58 aa, synthetic construct
  REGION 1..58: note = Modified bacterial sequence
VDAKYAKETIQAWDEIDRLPNLTLQQWLAFINKLDDDPSQSSELLSEAKKLNDSQAPK

SEQ ID NO: 737 - protein, 58 aa, synthetic construct
  REGION 1..58: note = Modified bacterial sequence
VDAKYAKETIQAWDEIDKLPNLTIEQWLAFINKLDDDPSQSSELLSEAKKLNDSQAPK

SEQ ID NO: 738 - protein, 58 aa, synthetic construct
  REGION 1..58: note = Modified bacterial sequence
VDAKYAKETLDAWAEIDHLPNLTIEQWLAFINKLDDDPSQSSELLSEAKKLNDSQAPK

SEQ ID NO: 739 - protein, 58 aa, synthetic construct
  REGION 1..58: note = Modified bacterial sequence
VDAKYAKEVIEAWDEIDKLPNLTLNQWLAFINKLDDDPSQSSELLSEAKKLNDSQAPK

SEQ ID NO: 740 - protein, 58 aa, synthetic construct
  REGION 1..58: note = Modified bacterial sequence
VDAKYAKEVLDAWNEIDQLPNLTIEQWLAFINKLDDDPSQSSELLSEAKKLNDSQAPK

SEQ ID NO: 741 - protein, 58 aa, synthetic construct
  REGION 1..58: note = Modified bacterial sequence
VDAKYAKEVLHAWNEIDHLPNLTIEQWLAFIEKLEDDPSQSSELLSEAKKLNDSQAPK

SEQ ID NO: 742 - protein, 58 aa, synthetic construct
  REGION 1..58: note = Modified bacterial sequence
VDAKYAKEVIEAWQEIDKLPNLTIDQWLAFINKLDDDPSQSSELLSEAKKLNDSQAPK

SEQ ID NO: 743 - protein, 58 aa, synthetic construct
  REGION 1..58: note = Modified bacterial sequence
VDAKYAKEVVDAWNEIDQLPNLTIEQWLAFINKLDDDPSQSSELLSEAKKLNDSQAPK

SEQ ID NO: 744 - protein, 58 aa, synthetic construct
  REGION 1..58: note = Modified bacterial sequence
VDAKYAKEQIEAWNEIDALPNLTIEQWLAFINKLADDPSQSSELLSEAKKLNDSQAPK

SEQ ID NO: 745 - protein, 60 aa, synthetic construct
  REGION 1..60: note = Modified bacterial sequence
VDAKYAKETITAWDEIDKLPNLTIEQWLAFIGKLEDDPSQSSELLAEAKKLNDAQAPKVD

SEQ ID NO: 746 - protein, 60 aa, synthetic construct
  REGION 1..60: note = Modified bacterial sequence
AEAKYAKEVIEAWNEIDRLPNLTIEQWLAFINKLDDDPSQSSELLSEAKKLNDSQAPKVD

SEQ ID NO: 747 - protein, 60 aa, synthetic construct
  REGION 1..60: note = Modified bacterial sequence
AEAKYAKEVLEAWNEIDRLPNLTIEQWLAFINKLDDDPSQSSELLSEAKKLNDSQAPKVD

SEQ ID NO: 748 - protein, 60 aa, synthetic construct
  REGION 1..60: note = Modified bacterial sequence
AEAKYAKEVLEAWDEIDRLPNLTLDQWLAFINKLDDDPSQSSELLSEAKKLNDSQAPKVD

SEQ ID NO: 749 - protein, 60 aa, synthetic construct
  REGION 1..60: note = Modified bacterial sequence
AEAKYAKEVLDAWDEIDKLPNLTLEQWLAFINKLDDDPSQSSELLSEAKKLNDSQAPKVD

SEQ ID NO: 750 - protein, 60 aa, synthetic construct
  REGION 1..60: note = Modified bacterial sequence
AEAKYAKEVLDAWDEIDALPNLTLEQWLAFINKLDDDPSQSSELLSEAKKLNDSQAPKVD

SEQ ID NO: 751 - protein, 60 aa, synthetic construct
  REGION 1..60: note = Modified bacterial sequence
AEAKYAKEVIDAWDEIDRLPNLTLDQWLAFINKLDDDPSQSSELLSEAKKLNDSQAPKVD

SEQ ID NO: 752 - protein, 60 aa, synthetic construct
  REGION 1..60: note = Modified bacterial sequence
AEAKYAKETLEAWDEIDRLPNLTIEQWLAFINKLDDDPSQSSELLSEAKKLNDSQAPKVD

SEQ ID NO: 753 - protein, 60 aa, synthetic construct
  REGION 1..60: note = Modified bacterial sequence
AEAKYAKEVLEAWDEIDRLPNLTIEQWLAFINKLDDDPSQSSELLSEAKKLNDSQAPKVD

SEQ ID NO: 754 - protein, 60 aa, synthetic construct
  REGION 1..60: note = Modified bacterial sequence
AEAKYAKEVIDAWNEIDALPNLTLDQWLAFINKLDDDPSQSSELLSEAKKLNDSQAPKVD

SEQ ID NO: 755 - protein, 60 aa, synthetic construct
  REGION 1..60: note = Modified bacterial sequence
AEAKYAKEVLDAWDEIDKLPNLTIDQWLAFINKLDDDPSQSSELLSEAKKLNDSQAPKVD

SEQ ID NO: 756 - protein, 60 aa, synthetic construct
  REGION 1..60: note = Modified bacterial sequence
AEAKYAKEVLEAWDEIDHLPNLTLDQWLAFINKLDDDPSQSSELLSEAKKLNDSQAPKVD

SEQ ID NO: 757 - protein, 60 aa, synthetic construct
  REGION 1..60: note = Modified bacterial sequence
AEAKYAKEVLEAWDEIDALPNLTIEQWLAFINKLDDDPSQSSELLSEAKKLNDSQAPKVD

SEQ ID NO: 758 - protein, 58 aa, synthetic construct [sequence omitted]

SEQ ID NO: 759 - protein, 46 aa, synthetic construct
  REGION 1..46: note = Modified bacterial sequence
LAEAKEAANAELDSYGVSDFYKRLIDKAKTVEGVEALKDAILAALP

SEQ ID NO: 760 - protein, 1676 aa, Homo sapiens
MGLLGILCFLIFLGKTWGQEQTYVISAPKIFRVGASENIVIQVYGYTEAFDATISIKSYPDKKFSYSSGHVHLSSENKFQNSAILTIQPKQLPGGQNPVSYVYLEVVSKHFSKSKRMPITYDNGFLFIHTDKPVYTPDQSVKVRVYSLNDDLKPAKRETVLTFIDPEGSEVDMVEEIDHIGIISFPDFKIPSNPRYGMWTIKAKYKEDFSTTGTAYFEVKEYVLPHFSVSIEPEYNFIGYKNFKNFEITIKARYFYNKVVTEADVYITFGIREDLKDDQKEMMQTAMQNTMLINGIAQVTFDSETAVKELSYYSLEDLNNKYLYIAVTVIESTGGFSEEAEIPGIKYVLSPYKLNLVATPLFLKPGIPYPIKVQVKDSLDQLVGGVPVTLNAQTIDVNQETSDLDPSKSVTRVDDGVASFVLNLPSGVTVLEFNVKTDAPDLPEENQAREGYRAIAYSSLSQSYLYIDWTDNHKALLVGEHLNIIVTPKSPYIDKITHYNYLILSKGKIIHFGTREKFSDASYQSINIPVTQNMVPSSRLLVYYIVTGEQTAELVSDSVWLNIEEKCGNQLQVHLSPDADAYSPGQTVSLNMATGMDSWVALAAVDSAVYGVQRGAKKPLERVFQFLEKSDLGCGAGGGLNNANVFHLAGLTFLTNANADDSQENDEPCKEILRPRRTLQKKIEEIAAKYKHSVVKKCCYDGACVNNDETCEQRAARISLGPRCIKAFTECCVVASQLRANISHKDMQLGRLHMKTLLPVSKPEIRSYFPESWLWEVHLVPRRKQLQFALPDSLTTWEIQGVGISNTGICVADTVKAKVFKDVFLEMNIPYSVVRGEQIQLKGTVYNYRTSGMQFCVKMSAVEGICTSESPVIDHQGTKSSKCVRQKVEGSSSHLVTFTVLPLEIGLHNINFSLETWFGKEILVKTLRVVPEGVKRESYSGVTLDPRGIYGTISRRKEFPYRIPLDLVPKTEIKRILSVKGLLVGEILSAVLSQEGINILTHLPKGSAEAELMSVVPVFYVFHYLETGNHWNIFHSDPLIEKQKLKKKLKEGMLSIMSYRNADYSYSVWKGGSASTWLTAFALRVLGQVNKYVEQNQNSICNSLLWLVENYQLDNGSFKENSQYQPIKLQGTLPVEARENSLYLTAFTVIGIRKAFDICPLVKIDTALIKADNFLLENTLPAQSTFTLAISAYALSLGDKTHPQFRSIVSALKREALVKGNPPIYRFWKDNLQHKDSSVPNTGTARMVETTAYALLTSLNLKDINYVNPVIKWLSEEQRYGGGFYSTQDTINAIEGLTEYSLLVKQLRLSMDIDVSYKHKGALHNYKMTDKNFLGRPVEVLLNDDLIVSTGFGSGLATVHVTTVVHKTSTSEEVCSFYLKIDTQDIEASHYRGYGNSDYKRIVACASYKPSREESSSGSSHAVMDISLPTGISANEEDLKALVEGVDQLFTDYQIKDGHVILQLNSIPSSDFLCVRFRIFELFEVGFLSPATFTVYEYHRPDKQCTMFYSTSNIKIQKVCEGAACKCVEADCGQMQEELDLTISAETRKQTACKPEIAYAYKVSITSITVENVFVKYKATLLDIYKTGEAVAEKDSEITFIKKVTCTNAELVKGRQYLIMGKEALQIKYNFSFRYIYPLDSLTWIEYWPRDTTCSSCQAFLANLDEFAEDIFLNGC

SEQ ID NO: 761 - protein, 170 aa, Ornithodoros moubata
MDSESDCTGSEPVDAFQAFSEGKEAYVLVRSTDPKARDCLKGEPAGEKQDNTLPVMMTFKNGTDWASTDWTFTLDGAKVTATLGNLTQNREVVYDSQSHHCHVDKVEKEVPDYEMWMLDAGGLEVEVECCRQKLEELASGRNQMYPHLKDCGGGGSENLYFQGSHHHHHH

SEQ ID NO: 762 - protein, 1676 aa, Macaca fascicularis
  SITE 63: note = misc_feature - Xaa can be any naturally occurring amino acid
  SITE 1346: note = misc_feature - Xaa can be any naturally occurring amino acid
MGLLGILCFLIFLGKTWGQEQTYVISAPKIFRVGASENIVIQVYGYTEAFDATISIKSYPDKXFSYSSGHVHLSSENKFQNSAVLTIQPKQLPGGQNQVSYVYLEVVSKHFSKSKKIPITYDNGFLFIHTDKPVYTPDQSVKVRVYSLNDDLKPAKRETVLTFIDPEGSEIDMVEEIDHIGIISFPDFKIPSNPRYGMWTIQAKYKEDFSTTGTAFFEVKEYVLPHFSVSVEPESNFIGYKNFKNFEITIKARIFYNKVVTEADVYITFGIREDLKDDQKEMMQTAMQNTMLINGIAEVTFDSETAVKELSYYSLEDLNNKYLYIAVTVIESTGGFSEEAEIPGIKYVLSPYKLNLVATPLFLKPGIPYSIKVQVKDALDQLVGGVPVTLNAQTIDVNQETSDLEPRKSVTRVDDGVASFVVNLPSGVTVLEFNVKTDAPDLPDENQAREGYRAIAYSSLSQSYLYIDWTDNHKALLVGEYLNIIVTPKSPYIDKITHYNYLILSKGKIIHFGTREKLSDASYQSINIPVTQNMVPSSRLLVYYIVTGEQTAELVSDSVWLNIEEKCGNQLQVHLSPDADTYSPGQTVSLNMVTGMDSWVALTAVDSAVYGVQRRAKKPLERVFQFLEKSDLGCGAGGGLNNANVFHLAGLTFLTNANADDSQENDEPCKEIIRPRRMLQEKIEEIAAKYKHLVVKKCCYDGVRINHDETCEQRAARISVGPRCVKAFTECCVVASQLRANNSHKDLQLGRLHMKTLLPVSKPEIRSYFPESWLWEVHLVPRRKQLQFALPDSVTTWEIQGVGISNSGICVADTIKAKVFKDVFLEMNIPYSVVRGEQVQLKGTVYNYRTSGMQFCVKMSAVEGICTSESPVIDHQGTKSSKCVRQKVEGSSNHLVTFTVLPLEIGLQNINFSLETSFGKEILVKSLRVVPEGVKRESYSGITLDPRGIYGTISRRKEFPYRIPLDLVPKTEIKRILSVKGLLVGEILSAVLSREGINILTHLPKGSAEAELMSVVPVFYVFHYLETGNHWNIFHSDPLIEKRNLEKKLKEGMVSIMSYRNADYSYSVWKGGSASTWLTAFALRVLGQVHKYVEQNQNSICNSLLWLVENYQLDNGSFKENSQYQPIKLQGTLPVEARENSLYLTAFTVIGIRKAFDICPLVKINTALIKADTFLLENTLPAQSTFTLAISAYALSLGDKTHPQFRSIVSALKREALVKGNPPIYRFWKDSLQHKDSSVPNTGTARMVETTAYALLTSLNLKDINYVNPIIKWLSEEQRYGGGFYSTQDTINAIEGLTEYSLLVKQLRLNMDIDVAYKHKGPLHNYKMTDKNFLGRPVEVLLNDDXVVSTGFGSGLATVHVTTVVHKTSTSEEVCSFYLKIDTQDVEASHYRGYGNSDYKRIVACASYKPSKEESSSGSSHAVMDISLPTGINANEEDLKALVEGVDQLFTDYQIKDGHVILQLNSIPSSDFLCVRFRIFELFEVGFLSPATFTVYEYHRPDKQCTMFYSTSNIKIQKVCEGATCKCIEADCGQMQKELDLTISAETRKQTACNPEIAYAYKVIITSITTENVFVKYKATLLDIYKTGEAVAEKDSEITFIKKVTCTNAELVKGRQYLIMGKEALQIKYNFTFRYIYPLDSLTWIEYWPRDTTCSSCQAFLANLDEFAEDIFLNGC

SEQ ID NO: 763 - protein, 12 aa, synthetic construct
  REGION 1..12: note = artificial
MGSSHHHHHHLQ

SEQ ID NO: 764 - DNA, 147 bp, synthetic construct
  misc_feature 1..147: note = artificial
  misc_feature 39..47: note = n is a, c, g, or t
  misc_feature 51..56: note = n is a, c, g, or t
  misc_feature 63..68: note = n is a, c, g, or t
  misc_feature 84..89: note = n is a, c, g, or t
  misc_feature 96..98: note = n is a, c, g, or t
  misc_feature 108..110: note = n is a, c, g, or t
  misc_feature 117..119: note = n is a, c, g, or t
  source 1..147: mol_type = other DNA
aaataaatctcgaggtagatgccaaatacgccaaagarnnnnnnnnngcmnnnnnngaratynnnnnnytrcctaacttaacynnnnnncartggnnngcsttcatynnnaarytrnnngaygacccaagccagagctcattattta

SEQ ID NO: 765 - protein, 12 aa, synthetic construct
  REGION 1..12: note = artificial
GSGGGGSGGGGS